European Patent Application EP 4 276 185 A2, published November 15, 2023. Title: NON-HUMAN ANIMALS COMPRISING A HUMANIZED TTR LOCUS AND METHODS OF USE. Applicant: Regeneron Pharmaceuticals, Inc. Application EP, filed September 28, 2018. The sequence listing filed with the application follows.

SEQUENCE LISTING (94 sequences)

SEQ ID NO: 1 - protein, 147 aa, Homo sapiens
MASHRLLLLCLAGLVFVSEAGPTGTGESKCPLMVKVLDAVRGSPAINVAVHVFRKAADDTWEPFASGKTSESGELHGLTTEEEFVEGIYKVEIDTKSYWKALGISPFHEHAEVVFTANDSGPRRYTIAALLSPYSYSTTAVVTNPKE

SEQ ID NO: 2 - protein, 147 aa, synthetic construct
  REGION 1..147: note = Synthetic
MASLRLFLLCLAGLVFVSEAGPAGTGESKCPLMVKVLDAVRGSPAINVAVHVFRKAADDTWEPFASGKTSESGELHGLTTEEEFVEGIYKVEIDTKSYWKALGISPFHEHAEVVFTANDSGPRRYTIAALLSPYSYSTTAVVTNPKE

SEQ ID NO: 3 - DNA, 7258 bp, Homo sapiens
  source 1..7258: mol_type = genomic DNA
gttgactaagtcaataatcagaatcagcaggtttgcagtcagattggcagggataagcagcctagctcaggagaagtgagtataaaagccccaggctgggagcagccatcacagaagtccactcattcttggcaggatggcttctcatcgtctgctcctcctctgccttgctggactggtatttgtgtctgaggctggccctacggtgagtgtttctgtgacatcccattcctacatttaagattcacgctaaatgaagtagaagtgactccttccagctttgccaaccagcttttattactagggcaagggtacccagcatctatttttaatataattaattcaaacttcaaaaagaatgaagttccactgagcttactgagctgggacttgaactctgagcattctacctcattgctttggtgcattaggtttgtaatatctggtacctctgtttcctcagatagatgatagaaataaagatatgatattaaggaagctgttaatactgaattttcagaaaagtatccctccataaaatgtatttgggggacaaactgcaggagattatattctggccctatagttattcaaaacgtatttattgattaatctttaaaaggcttagtgaacaatattctagtcagatatctaattcttaaatcctctagaagaattaactaatactataaaatgggtctggatgtagttctgacattattttataacaactggtaagagggagtgactatagcaacaactaaaatgatctcaggaaaacctgtttggccctatgtatggtacattacatcttttcagtaattccactcaaatggagacttttaacaaagcaactgttctcaggggacctattttctcccttaaaattcattatacacatccctggttgatagcagtgtgtctggaggcagaaaccattcttgctttggaaacaattacgtctgtgttatactgagtagggaagctcattaattgtcgacacttacgttcctgataatgggatcagtgtgtaattcttgtttcgctccagatttctaataccacaaagaataaatcctttcactctgatcaattttgttaacttctcacgtgtcttctctacacccagggcaccggtgaatccaagtgtcctctgatggtcaaagttctagatgctgtccgaggcagtcctgccatcaatgtggccgtgcatgtgttcagaaaggctgctgatgacacctgggagccatttgcctctgggtaagttgccaaagaaccctcccacaggacttggttttatcttcccgtttgcccctcacttggtagagagaggctcacatcatctgctaaagaatttacaagtagattgaaaaacgtaggcagaggtcaagtatgccctctgaaggatgccctctttttgttttgcttagctaggaagtgaccaggaacctgagcatcatttaggggcagacagtagagaaaagaaggaatcagaactcctctcctctagctgtggtttgcaacccttttgggtcacagaacactttatgtaggtgatgaaaagtaaacattctatgcccagaaaaaatgcacagatacacacacatacaaaatcatatatgtgattttaggagtttcacagattccctggtgtccctgggtaacaccaaagctaagtgtccttgtcttagaattttaggaaaaggtataatgtgtattaacccattaacaaaaggaaaggaattcagaaatattattaaccaggcatctgtctgtagttaatatggatcacccaaaacccaaggcttttgcctaatgaacactttggggcacctactgtgtgcaaggctgggggctgtcaagctcagttaaaaaaaaaaagatagaagagatggatccatgaggcaaagtacagccccaggctaatcccacgatcacccgacttcatgtccaagagtggcttctcaccttcattagccagttcacaattttcatggagtttttctacctgcactagcaaaaacttcaaggaaaatacatattaataaatctaagcaaagtgaccagaagacagagcaatcaggagaccctttgcatccagcagaagaggaactgctaagtatttacatctccacagagaagaatttctgttgggttttaattgaaccccaagaaccacatgattcttcaaccattattgggaagatcattttcttaggtctggttttaactggctttttatttgggaattcatttatgtttatataaaatgccaagcataacatgaaaagtggttacaggactattctaagggagagacagaatggacaccaaaaatattccaatgttcttgtgaatcttttccttgcaccaggacaaaaaaaaaaagaagtgaaaagaagaaaggaggaggggcataatcagagtcagtaaagacaactgctatttttatctatcgtagctgttgcagtcaaatgggaagcaatttccaacattcaactatggagctggtacttacatggaaatagaagttgcctagtgtttgttgctggcaaagagttatcagagaggttaaatatataaaagggaaaagagtcagatacaggttcttcttcctactttaggttttccactgtgtgtgcaaatgatactccctggtggtgtgcagatgcctcaaagctatcctcacaccacaagggagaggagcgagatcctgctgtcctggagaagtgcagagttagaacagctgtggccacttgcatccaatcatcaatcttgaatcacagggactctttcttaagtaaacattatacctggccgggcacggtggctcacgcctgtaatcccagcactttgggatgccaaagtgggcatatcatctgaggtcaggagttcaagaccagcctggccaacatggcaaaactccgtctttatgaaaaatacaaaaattagccaggcatggtggcaggcgcctgtaatcccagctaattgggaggctgaggctggagaatcccttgaatctaggaggcagaggttgcagtgagctgagatcgtgccattgcactccagcctgggtgacaagagtaaaactctgtctcaaaaaaaaaaaattatacctacattctcttcttatcagagaaaaaaatctacagtgagcttttcaaaaagtttttacaaactttttgccatttaatttcagttaggagttttccctacttctgacttagttgaggggaaatgttcataacatgtttataacatgtttatgtgtgttagttggtgggggtgtattactttgccatgccatttgtttcctccatgcgtaacttaatccagactttcacaccttataggaaaaccagtgagtctggagagctgcatgggctcacaactgaggaggaatttgtagaagggatatacaaagtggaaatagacaccaaatcttactggaaggcacttggcatctccccattccatgagcatgcagaggtgagtatacagaccttcgagggttgttttggttttggtttttgcttttggcattccaggaaatgcacagttttactcagtgtaccacagaaatgtcctaaggaaggtgatgaatgaccaaaggttccctttcctattatacaagaaaaaattcacaacactctgagaagcaaatttctttttgactttgatgaaaatccacttagtaacatgacttgaacttacatgaaactactcatagtctattcattccactttatatgaatattgatgtatctgctgttgaaataatagtttatgaggcagccctccagaccccacgtagagtgtatgtaacaagagatgcaccattttatttctcgaaaacccgtaacattcttcattccaaaacacatctggcttctcggaggtctggacaagtgattcttggcaacacatacctatagagacaataaaatcaaagtaataatggcaacacaatagataacatttaccaagcatacaccatgtggcagacacaattataagtgttttccatatttaacctacttaatcctcaggaataagccactgaggtcagtcctattattatccccatcttatagatgaagaaaatgaggcaccaggaagtcaaataacttgtcaaaggtcacaagactaggaaatacacaagtagaaatgtttacaattaaggcccaggctgggtttgccctcagttctgctatgcctcgcattatgccccaggaaactttttcccttgtgaaagccaagcttaaaaaaagaaaagccacatttgtaacgtgctctgttcccctgcctatggtgaggatcttcaaacagttatacatggacccagtccccctgccttctccttaatttcttaagtcatttgaaacagatggctgtcatggaaatagaatccagacatgttggtcagagttaaagatcaactaattccatcaaaaatagctcggcatgaaagggaactattctctggcttagtcatggatgagactttcaattgctataaagtggttcctttattagacaatgttaccagggaaacaacaggggtttgtttgacttctggggcccacaagtcaacaagagagccccatctaccaaggagcatgtccctgactacccctcagccagcagcaagacatggaccccagtcagggcaggagcagggtttcggcggcgcccagcacaagacattgcccctagagtctcagcccctaccctcgagtaatagatctgcctacctgagactgttgtttgcccaagagctgggtctcagcctgatgggaaccatataaaaaggttcactgacatactgcccacatgttgttctctttcattagatcttagcttccttgtctgctcttcattcttgcagtattcattcaacaaacattaaaaaaaaaaaaaagcattctatgtgtggaacactctgctagatgctgtggatttagaaatgaaaatacatcccgacccttggaatggaagggaaaggactgaagtaagacagattaagcaggaccgtcagcccagcttgaagcccagataaatacggagaacaagagagagcgagtagtgagagatgagtcccaatgcctcactttggtgacgggtgcgtggtgggcttcatgcagcttcttctgataaatgcctccttcagaactggtcaactctaccttggccagtgacccaggtggtcatagtagatttaccaagggaaaatggaaacttttattaggagctcttaggcctcttcacttcatggatttttttttcctttttttttgagatggagttttgccctgtcacccaggctggaatgcagtggtgcaatctcagctcactgcaacctccgcctcccaggttcaagcaattctcctgcctcagcctcccgagtagctgggactacaggtgtgcgccaccacaccaggctaatttttgtattttttgtaaagacaggttttcaccacgttggccaggctggtctgaactccagacctcaggtgattcacctgtctcagcctcccaaagtgctgggattacaggtgtgagccaccgtgcccggctacttcatggatttttgattacagattatgcctcttacaatttttaagaagaatcaagtgggctgaaggtcaatgtcaccataagacaaaagacatttttattagttgattctagggaattggccttaaggggagccctttcttcctaagagattcttaggtgattctcacttcctcttgccccagtattatttttgtttttggtatggctcactcagatccttttttcctcctatccctaagtaatccgggtttctttttcccatatttagaacaaaatgtatttatgcagagtgtgtccaaacctcaacccaaggcctgtatacaaaataaatcaaattaaacacatctttactgtcttctacctctttcctgacctcaatatatcccaacttgcctcactctgagaaccaaggctgtcccagcacctgagtcgcagatattctactgatttgacagaactgtgtgactatctggaacagcattttgatccacaatttgcccagttacaaagcttaaatgagctctagtgcatgcatatatatttcaaaattccaccatgatcttccacactctgtattgtaaatagagccctgtaatgcttttacttcgtatttcattgcttgttatacataaaaatatacttttcttcttcatgttagaaaatgcaaagaataggagggtgggggaatctctgggcttggagacaggagacttgccttcctactatggttccatcagaatgtagactgggacaatacaataattcaagtctggtttgctcatctgtaaattgggaagaatgtttccagctccagaatgctaaatctctaagtctgtggttggcagccactattgcagcagctcttcaatgactcaatgcagttttgcattctccctaccttttttttctaaaaccaataaaatagatacagcctttaggctttctgggatttcccttagtcaagctagggtcatcctgactttcggcgtgaatttgcaaaacaagacctgactctgtactcctgctctaaggactgtgcatggttccaaaggcttagcttgccagcatatttgagctttttccttctgttcaaactgttccaaaatataaaagaataaaattaattaagttggcactggacttccggtggtcagtcatgtgtgtcatctgtcacgtttttcgggctctggtggaaatggatctgtctgtcttctctcataggtggtattcacagccaacgactccggcccccgccgctacaccattgccgccctgctgagcccctactcctattccaccacggctgtcgtcaccaatcccaaggaatgagggacttctcctccagtggacctgaaggacgagggatgggatttcatgtaaccaagagtattccatttttactaaagcagtgttttcacctcatatgctatgttagaagtccaggcagagacaataaaacattcctgtgaaaggcacttttcattccactttaacttgattttttaaattcccttattgtcccttccaaaaaaaagagaatcaaaattttacaaagaatcaaaggaattctagaaagtatctgggcagaacgctaggagagatccaaatttccattgtcttgcaagcaaagcacgtattaaatatgatctgcagccattaaaaagacacattctgtaaa

SEQ ID NO: 4 - DNA, 938 bp, Homo sapiens
  source 1..938: mol_type = other DNA
gttgactaagtcaataatcagaatcagcaggtttgcagtcagattggcagggataagcagcctagctcaggagaagtgagtataaaagccccaggctgggagcagccatcacagaagtccactcattcttggcaggatggcttctcatcgtctgctcctcctctgccttgctggactggtatttgtgtctgaggctggccctacgggcaccggtgaatccaagtgtcctctgatggtcaaagttctagatgctgtccgaggcagtcctgccatcaatgtggccgtgcatgtgttcagaaaggctgctgatgacacctgggagccatttgcctctgggaaaaccagtgagtctggagagctgcatgggctcacaactgaggaggaatttgtagaagggatatacaaagtggaaatagacaccaaatcttactggaaggcacttggcatctccccattccatgagcatgcagaggtggtattcacagccaacgactccggcccccgccgctacaccattgccgccctgctgagcccctactcctattccaccacggctgtcgtcaccaatcccaaggaatgagggacttctcctccagtggacctgaaggacgagggatgggatttcatgtaaccaagagtattccatttttactaaagcagtgttttcacctcatatgctatgttagaagtccaggcagagacaataaaacattcctgtgaaaggcacttttcattccactttaacttgattttttaaattcccttattgtcccttccaaaaaaaagagaatcaaaattttacaaagaatcaaaggaattctagaaagtatctgggcagaacgctaggagagatccaaatttccattgtcttgcaagcaaagcacgtattaaatatgatctgcagccattaaaaagacacattctgtaaaaaaaaaaaa

SEQ ID NO: 5 - DNA, 9077 bp, Mus musculus
  source 1..9077: mol_type = genomic DNA
ctaatctccctaggcaaggttcatatttgtgtaggttacttattctccttttgttgactaagtcaataatcagaatcagcaggtttggagtcagcttggcagggatcagcagcctgggttggaaggagggggtataaaagccccttcaccaggagaagccgtcacacagatccacaagctcctgacaggatggcttcccttcgactcttcctcctttgcctcgctggactggtatttgtgtctgaagctggccccgcggtgagtgatcctgtgagcgatccagacatggcagttagaccttagataaagaagaagtgccttcttccagatgtgagaactagagtactcagactctatatttaccattagactccaaagagaagagctggagtgcctctggctcttccttctattgctttagcgcattgggtctgtagtgctcagtctctggtgtccttagataataaagatatgagattaacatagaaataaagatataaaagggctggatgtatagtttagtggtccagtgtatgcctagtatgtgaaaagccttctgttcaacctctagcaatagaaaaacaagatatattctcggtggggctgttaatattgaattctcataaaatctttaatatatttagtatgcctattatgttgttatattttagttctttagctaatcaaaatgcattattgatctttctttgtctttttttggccaacactctattccagtctttgaaaaagtcctttaaaagagttaatcagtataattaaatgagtcaggaagtatgtgagggttattttacaaccagagggaattactatagcaacagctgattagaatgatctcaagaaaaagcccattctgtctttttgcaccatgcacctttcagtggctccattcagatggagaggcaaacagagcaatggctctcagagggcctattttccctttgaacattcattatccatatccctggtgcacagcagtgcatctgggggcagaaactgttcttgctttggaaacaatgctgtctatgtcatactggataaagaagctcattaattgtcaacacttatgttatcataatgggatcagcatgtacttttggttttgttccagagtctatcaccggaaagaacaagccggtttactctgacccatttcactgacatttctcttgtctcctctgtgcccagggtgctggagaatccaaatgtcctctgatggtcaaagtcctggatgctgtccgaggcagccctgctgtagacgtggctgtaaaagtgttcaaaaagacctctgagggatcctgggagccctttgcctctgggtaagcttgtagaaagcccaccatgggaccggttccaggttcccatttgctcttattcgtgttagattcagacacacacaacttaccagctagagggctcagagagagggctcaggggcgaagggcacgtattgctcttgtaagagacacaggtttaattcctagcaccagaatggcagctcataaccatctgaaactcacagtcttaggagatctgggtatctgacattctcttctacccaccatgtgtgtggtgcacaaattcacatgcaggcatcaaatcttataaacaacaacaaaaaaccaacaaacctggtagcaaaagaagattagaaggttaaacatatgagccgagagcttttgttttgttttgttttgttttgttttgtttacatttcaaatgttatcccctttctcggtccccctccccaaaccctctaccccattctctcctccccttcttctatgagggtgttccccaccaacccactcccaccttcctgctctcgaattcccctatactgggacatcaagccttcacagaatcaagggcctctcctcccattgatgcccgacaatgtcatcctctgctacctatgtggctggagccatgggtcccttcatgtatcctccttggttggtggtttagtctctgggaggtctgggggatctggttgattgatattattgttcttcctatgagattgcaaaccccttcagctccttcggtcctttaactcctccactggggaccccgagctcagtccaatggttggctgtgagcatccaccagcagaggcctttttttttttttttaacaaagctgctttattatgttgcttagagcatgaccaggaaccagagcacagtccaagactgaagggaggaaaagggggggagtcaataaccccactgtttcatagtggtttgcaacccttttatatcacagcccactttaggcaaataatgaaaattatagtctccagggacagagaagatggtgcaggaagtgaagtgcctgctcagaaaatgggggcttgaatgtgagttcccagactctgtgtaagatgcccagcatcgaagtgcatgcttataacaccagcctggaggtagaagcttagaaacaggggtaccctgaagttgcttgttcaccagtgtccctgaatgggtaggtgcatgtttggtgagagaccctgtctcaaaaatcaaggtgtaggataattgaaaatacctagctttgagcttagatcatgcaaatgtgtacacacactcacacacaccacacacacaaaaaaatgcagagacagagagatacagagagacagagagatacagagacagagacagagagaaaaggagaaagtaaaaaacaaataatttaaagacccatggccacaaagaggctcaaagacaagcacgtataaaaccatacacatgtaattttaggagttttcagattccctggtacccgtgggtgatgcacaagctttgaatcccagtcttaaaatcttacgaagaacgtgttcgtgtgtgctaatttattgatgagaggaaaggaattgacaaagtgcccttccggagcttcctgcattacccagactcagggtttttttaaatgtacactcagaacagagtagctctgtgcaagggtagcaaccacgaagcttaataagaaacatatcgtgagagatctgcaaggcaaatctaggggctgaccaatctcacagtcacccactagcatgtcaacacaacttcccacctgtgctagccacttagcaattttgtgttgttctgttttgtttttgtttttaacaaagcaatttcaaagagatttctaattcatctaaacaaacaaaccaaaaggaaaacagcaaagacgccctgagcacttagcagagcagctatgcagttatgactcctgggtggagactttatatcaggcttcaactgaatacctagaacctactagtgctcttcatcaatccttgggaaggtcattttcttttggtgctgttttgagtttctatttgttaatgtcttcataattatacacgtgttgagcacagcatgcaaagtgattaggggaatctagttggagtggaatggatacccaaatattcagactttcttgtgactcttctttcttgtacccacatcaaaaaaaaaaaaaatggagatgagacatggtcagagtcactaaaaccagctgctacttttaattacgtggggagcagtttctaacattgccattattgaactgatgctgcctgggtggaaatggaaatcacttagtatttcttgttggcaaagaattactgaatggattaaatttccaaagggagaagtcagttacaagtcttttctttgtttattaggctttctgctatgataaattacactacttccagaagttacccttaggccatgggacactggactatcactctgctgtcacaagagattacagagttagtcaaggcagcttgtgacaccttcagggactgtcataaacttccagcaagtcattaatcctgaatgcaatactgtgtgtgtgtgtctatgtgtgtttgtatgtctgtgtgtgtcttatgtctgtgtctctgtgtgtgtgtgtgtttgtgtgtgtgtgtgtatgtatgcctgtgtgtgtcttatgtctgtgtttgtgtgtctgtgtgtgtcttatgtctgtgtttgtatgtctgtgtgtgtctgtgtgtgtcttatgtctgtgtctctgtgtgtgtgtgtgtgtatgtatgtatgtatgtatgtatgtgtatgtgtttgcatctctctgtgtgtctgcgcttatatatttgtgtatgtgtttatgtgttcgcctttgtgcgttgttggggattgaatccaggggaatacaaatgttaagaaagaacgttaccactaagcttcacctgtaggccttaaagcttttctttcttttaaaaattgtaattaattcattttcagtcaggatctccacacctcgtccctgctgctctagaactcactatttaaacacaatcgccctcaaacctgcagcaaccctcccgcctctaccctgcgagcactagaataataacaggtgaccccacacgcctagattaagacctttaaggtaaacattttactatattttagtctcataagacaagatgctacaataaagctgtacataaagttccctcgaatttcttgctattttaactcaaacataaggatttcctcctttttgattcaggtaacagaaaaaatacacaggtacatacatgtacacacatgaacacacacgcatcacaaccacatatgcgcacgcttgtgtgatctatcatttaccatgccactgaactcttctttccccataaattcctctggacttgtgtgccctccaggaagaccgcggagtctggagagctgcacgggctcaccacagatgagaagtttgtagaaggagtgtacagagtagaactggacaccaaatcgtactggaagacacttggcatttccccgttccatgaattcgcggatgtaagtggacacaccaagttgtttggattttgtttttagtctcaggaaattcccttcgctcttgctgtacgatgggcatgagtggaaagtagattccacagccagaatccacagtgctgggaaagcaagccttctgaatttttctaaaactcatttagcaacatggcctgaacctgttcacactgcttatggtcagctaactatatttatgtaaatattcatttctctgttgaggaaatgttagtatttgcttttgaggcaacctccagataccatggagggcatgtcatagtcaaagagagggctccctatggtatttctctaaattctggcatttcctttattccaaagcacatctagtgtccccagaagtttgggtagacaattcttggcaacacagagaattacaacatgttcaaaacccaacagcttaatatctaaatcatcaagcaaacatcacatggcaaagggatttctgaatcaaaactgtttcatccttatgatcaacctatggaggtctagcctcgacttacacccattttaccaataagctaagagaagctaagttcctcatcaaggacacaaggctagcatgtgtgagcaagtgacagagttgccctctatgttggttagtgtgccttagccagtgtctcagtaagaaatggagctaaatcaaaacccaaggccaacagccaaaggcacatgagtaacctttgcttggcactgggctcagtttccctggctcctctcagtcctcagttcacagaggcagctgtcatgcaaatagaatccaagcttgttggtcagacctggagataacaaattccatcaaaaatagctcctcatgtgacctagtttgctgtctgttgctatgatacacaccatgaccgaaaagcaaccctggggagagaagggtttatttcatcttacagcttacagttcaccatggaggaaagccaggtgggaacctggaagtggaaattgaagcagagaccagaaaggaatgctgtttactggctggcttagctccttttcttatacagcttaggtctatgtgcccaggggatggtactgccgagcataggctgagcccgcctacatcaaccattagtcaaaaaaaggtccatagacttgcctacaggccaatctcatggaggcaataccccagtggagggtccctcttcgcaggttactctagtttgtgtcaagttgacaaaacctaaccacaaagcacaaacagggtctgcccttgtggcttagccatggatgacactctcagatgatggtgttaccagacaaaccagaggggctcaccaagagtctgccacctaccaaggtagtactctactcctcactgggcaccaacacccatattagctgggccagtacaggacccttgctgtttcctgcatgaattgtccatagaccctgggtctcagcctgccgggagtacctgtaagtagtcgcctcaaacacattattcctgttggaagacttgtctgattctcttttagaactcaatcaacaaacgtttttattttgttttggctttttggagacaagatctctcataggccagcctgacttgaatgtagctgaggatgacctgtgctgctaatcttctcgcctcttcctcccaagtggtaggataataggcataagacaccacagcagttttactccataccagggctctgaacccagactttaaacactctatcaactgattcacattcccaccccatcattcaacaaacatttgaaaaataaaacccttctgccttgagcactctgctaaatacagcctttgagtgcggagtatttcctcacaaccagggtccaagatgaccccatcatacataccacggaaaattaggagatgtttttaggtctctttgcttggggtaatttttatgtgtgtgtgtacacagccctgtgcgtgtgtgtgtgtgtgtgtgtgtgtgtgtacaggcacacacgtgtatgcatgtagaggctacataaaaaccttaggtgtcattctcaggcactctgttcaccccttcacacagcccgaacacacaaaatttgaggcattagcctggagctcaccagttaggctagactgacttgccagcagaccccaggctgtctccatctccccagctctgggattacaaactctatcataccagacatttttatacatattctgagcataaaattcatgtcttcaggctaacaagtcaagagcttaaatgactgagctctcttacgtggtggattttttttaaaactacataatatcttttttttttttttcacttctggggaagaaacaaatgagcctgagtgacaatgcgacagaaaagaaattttgaggagtgtgtgtgtctgtgtgtgtggtggcacatgcctctcatctaatgctagaggctacagtagaatgctcctgaattagtggccagccaaggccaagggctagggttgtaactcagtggcagagggcttgcctagcattcgcaggatttgatccatagcgctataaataataataaataaatacaacagtctaagatgattctccctttcatttatctggatgttatttttgtgttagttttactctgtcatccaatcattgtttgccctatatttggacatttaaaaaaaatctttattccaagtgtgttcaaagctgtatccaaaacctgtccaccaaatgagtccaatgacatacatcttctatattaccatctgttccagatttggctgactcccggcacctgggctgttgctgcacccatgtctcagatagtctagtgatttgagaagtgactagtaattgcaaaatccagactttgtccagaaacttctatgagctccaaaactttcatttacatttctgccagccacaaaccgcttgtgttgtggagagaaccctgtgatgtcttcccacagcatctcagccttgtttcttcccttaaaatattcatcttttcacattagaacatgcaaagggacagtgggagcgaaacccctggactgggacgcacgaagccttcctttctggtcaggctctcactgtagaaacttaggccggtttcagcatgcagtctgctggagaatggctcctgccaacattccaggtctggaagtttgtagtggagttgttgataaccactgttcgccacaggtcttttgtttgtgggtgtcagtgtttctactctcctgacttttatctgaacccaagaaagggaacaatagccttcaagctctctgtgactctgatctgaccagggccacccacactgcagaaggaaacttgcaaagagagacctgcaattctctaagagctccacacagctccaaagacttaggcagcatattttaatctaattattcgtcccccaaccccaccccagaggacagttagacaataaaaggaagattaccagcttagcatcctgtgaacactttgtctgcagctcctacctctgggctctgttagaactagctgtctctcctctctcctaggtggttttcacagccaacgactctggccatcgccactacaccatcgcagccctgctcagcccatactcctacagcaccacggctgtcgtcagcaacccccagaattgagagactcagcccaggaggaccaggatcttgccaaagcagtagcatcccatttgtaccaaaacagtgttcttgctctataaaccgtgttagcagctcaggaagatgccgtgaagcattcttattaaaccacctgctatttcattcaaactgtgtttcttttttatttcctcatttttctcccctgctcctaaaacccaaaatcttctaaagaattctagaaggtatgcgatcaaactttttaaagaaagaaaatactttttgactcatggtttaaaggcatcctttccatcttggggaggtcatgggtgctcctggcaacttgcttgaggaagataggtcagaaagcagagtggaccaaccgttcaatgttttacaagcaaaacatacactaagcatggtctgtagctattaaaagcacacaatctgaagggctgtagatgcacagtagtgttttcccagagcatgttcaaaagccctgggttcaatcacaatactgaaaagtaggccaaaaaacattctgaaaatgaaatatttgggtttttttttataacctttagtgactaaataaagacaaatctaagagactaa

SEQ ID NO: 6 - protein, 147 aa, Mus musculus
MASLRLFLLCLAGLVFVSEAGPAGAGESKCPLMVKVLDAVRGSPAVDVAVKVFKKTSEGSWEPFASGKTAESGELHGLTTDEKFVEGVYRVELDTKSYWKTLGISPFHEFADVVFTANDSGHRHYTIAALLSPYSYSTTAVVSNPQN

SEQ ID NO: 7 - DNA, 1237 bp, Mus musculus
  source 1..1237: mol_type = other DNA
ctaatctccctaggcaaggttcatatttgtgtaggttacttattctccttttgttgactaagtcaataatcagaatcagcaggtttggagtcagcttggcagggatcagcagcctgggttggaaggagggggtataaaagccccttcaccaggagaagccgtcacacagatccacaagctcctgacaggatggcttcccttcgactcttcctcctttgcctcgctggactggtatttgtgtctgaagctggccccgcgggtgctggagaatccaaatgtcctctgatggtcaaagtcctggatgctgtccgaggcagccctgctgtagacgtggctgtaaaagtgttcaaaaagacctctgagggatcctgggagccctttgcctctgggaagaccgcggagtctggagagctgcacgggctcaccacagatgagaagtttgtagaaggagtgtacagagtagaactggacaccaaatcgtactggaagacacttggcatttccccgttccatgaattcgcggatgtggttttcacagccaacgactctggccatcgccactacaccatcgcagccctgctcagcccatactcctacagcaccacggctgtcgtcagcaacccccagaattgagagactcagcccaggaggaccaggatcttgccaaagcagtagcatcccatttgtaccaaaacagtgttcttgctctataaaccgtgttagcagctcaggaagatgccgtgaagcattcttattaaaccacctgctatttcattcaaactgtgtttcttttttatttcctcatttttctcccctgctcctaaaacccaaaatcttctaaagaattctagaaggtatgcgatcaaactttttaaagaaagaaaatactttttgactcatggtttaaaggcatcctttccatcttggggaggtcatgggtgctcctggcaacttgcttgaggaagataggtcagaaagcagagtggaccaaccgttcaatgttttacaagcaaaacatacactaagcatggtctgtagctattaaaagcacacaatctgaagggctgtagatgcacagtagtgttttcccagagcatgttcaaaagccctgggttcaatcacaatactgaaaagtaggccaaaaaacattctgaaaatgaaatatttgggtttttttttataacctttagtgactaaataaagacaaatctaagagactaaaaaaaaaaaaaaaaaa

SEQ ID NO: 8 - RNA, 82 nt, synthetic construct
  misc_feature 1..82: note = Synthetic
  source 1..82: mol_type = other RNA
gttggaaccattcaaaacagcatagcaagttaaaataaggctagtccgttatcaacttgaaaaagtggcaccgagtcggtgc

SEQ ID NO: 9 - RNA, 76 nt, synthetic construct
  misc_feature 1..76: note = Synthetic
  source 1..76: mol_type = other RNA
gttttagagctagaaatagcaagttaaaataaggctagtccgttatcaacttgaaaaagtggcaccgagtcggtgc

SEQ ID NO: 10 - RNA, 86 nt, synthetic construct
  misc_feature 1..86: note = Synthetic
  source 1..86: mol_type = other RNA
gtttaagagctatgctggaaacagcatagcaagtttaaataaggctagtccgttatcaacttgaaaaagtggcaccgagtcggtgc

SEQ ID NO: 11-13 - skipped (3 entries)

SEQ ID NO: 14 - DNA, 12208 bp, synthetic construct
  misc_feature 1..12208: note = Synthetic
  misc_feature 1..97: note = Mouse Sequence
  misc_feature 98..7298: note = Human Sequence
  misc_feature 7299..12108: note = SDC Neo Cassette
  misc_feature 12109..12208: note = Mouse Sequence
  source 1..12208: mol_type = other DNA
agcttggcagggatcagcagcctgggttggaaggagggggtataaaagccccttcaccaggagaagccgtcacacagatccacaagctcctgacaggatggcttctcatcgtctgctcctcctctgccttgctggactggtatttgtgtctgaggctggccctacggtgagtgtttctgtgacatcccattcctacatttaagattcacgctaaatgaagtagaagtgactccttccagctttgccaaccagcttttattactagggcaagggtacccagcatctatttttaatataattaattcaaacttcaaaaagaatgaagttccactgagcttactgagctgggacttgaactctgagcattctacctcattgctttggtgcattaggtttgtaatatctggtacctctgtttcctcagatagatgatagaaataaagatatgatattaaggaagctgttaatactgaattttcagaaaagtatccctccataaaatgtatttgggggacaaactgcaggagattatattctggccctatagttattcaaaacgtatttattgattaatctttaaaaggcttagtgaacaatattctagtcagatatctaattcttaaatcctctagaagaattaactaatactataaaatgggtctggatgtagttctgacattattttataacaactggtaagagggagtgactatagcaacaactaaaatgatctcaggaaaacctgtttggccctatgtatggtacattacatcttttcagtaattccactcaaatggagacttttaacaaagcaactgttctcaggggacctattttctcccttaaaattcattatacacatccctggttgatagcagtgtgtctggaggcagaaaccattcttgctttggaaacaattacgtctgtgttatactgagtagggaagctcattaattgtcgacacttacgttcctgataatgggatcagtgtgtaattcttgtttcgctccagatttctaataccacaaagaataaatcctttcactctgatcaattttgttaacttctcacgtgtcttctctacacccagggcaccggtgaatccaagtgtcctctgatggtcaaagttctagatgctgtccgaggcagtcctgccatcaatgtggccgtgcatgtgttcagaaaggctgctgatgacacctgggagccatttgcctctgggtaagttgccaaagaaccctcccacaggacttggttttatcttcccgtttgcccctcacttggtagagagaggctcacatcatctgctaaagaatttacaagtagattgaaaaacgtaggcagaggtcaagtatgccctctgaaggatgccctctttttgttttgcttagctaggaagtgaccaggaacctgagcatcatttaggggcagacagtagagaaaagaaggaatcagaactcctctcctctagctgtggtttgcaacccttttgggtcacagaacactttatgtaggtgatgaaaagtaaacattctatgcccagaaaaaatgcacagatacacacacatacaaaatcatatatgtgattttaggagtttcacagattccctggtgtccctgggtaacaccaaagctaagtgtccttgtcttagaattttaggaaaaggtataatgtgtattaacccattaacaaaaggaaaggaattcagaaatattattaaccaggcatctgtctgtagttaatatggatcacccaaaacccaaggcttttgcctaatgaacactttggggcacctactgtgtgcaaggctgggggctgtcaagctcagttaaaaaaaaaaagatagaagagatggatccatgaggcaaagtacagccccaggctaatcccacgatcacccgacttcatgtccaagagtggcttctcaccttcattagccagttcacaattttcatggagtttttctacctgcactagcaaaaacttcaaggaaaatacatattaataaatctaagcaaagtgaccagaagacagagcaatcaggagaccctttgcatccagcagaagaggaactgctaagtatttacatctccacagagaagaatttctgttgggttttaattgaaccccaagaaccacatgattcttcaaccattattgggaagatcattttcttaggtctggttttaactggctttttatttgggaattcatttatgtttatataaaatgccaagcataacatgaaaagtggttacaggactattctaagggagagacagaatggacaccaaaaatattccaatgttcttgtgaatcttttccttgcaccaggacaaaaaaaaaaagaagtgaaaagaagaaaggaggaggggcataatcagagtcagtaaagacaactgctatttttatctatcgtagctgttgcagtcaaatgggaagcaatttccaacattcaactatggagctggtacttacatggaaatagaagttgcctagtgtttgttgctggcaaagagttatcagagaggttaaatatataaaagggaaaagagtcagatacaggttcttcttcctactttaggttttccactgtgtgtgcaaatgatactccctggtggtgtgcagatgcctcaaagctatcctcacaccacaagggagaggagcgagatcctgctgtcctggagaagtgcagagttagaacagctgtggccacttgcatccaatcatcaatcttgaatcacagggactctttcttaagtaaacattatacctggccgggcacggtggctcacgcctgtaatcccagcactttgggatgccaaagtgggcatatcatctgaggtcaggagttcaagaccagcctggccaacatggcaaaactccgtctttatgaaaaatacaaaaattagccaggcatggtggcaggcgcctgtaatcccagctaattgggaggctgaggctggagaatcccttgaatctaggaggcagaggttgcagtgagctgagatcgtgccattgcactccagcctgggtgacaagagtaaaactctgtctcaaaaaaaaaaaattatacctacattctcttcttatcagagaaaaaaatctacagtgagcttttcaaaaagtttttacaaactttttgccatttaatttcagttaggagttttccctacttctgacttagttgaggggaaatgttcataacatgtttataacatgtttatgtgtgttagttggtgggggtgtattactttgccatgccatttgtttcctccatgcgtaacttaatccagactttcacaccttataggaaaaccagtgagtctggagagctgcatgggctcacaactgaggaggaatttgtagaagggatatacaaagtggaaatagacaccaaatcttactggaaggcacttggcatctccccattccatgagcatgcagaggtgagtatacagaccttcgagggttgttttggttttggtttttgcttttggcattccaggaaatgcacagttttactcagtgtaccacagaaatgtcctaaggaaggtgatgaatgaccaaaggttccctttcctattatacaagaaaaaattcacaacactctgagaagcaaatttctttttgactttgatgaaaatccacttagtaacatgacttgaacttacatgaaactactcatagtctattcattccactttatatgaatattgatgtatctgctgttgaaataatagtttatgaggcagccctccagaccccacgtagagtgtatgtaacaagagatgcaccattttatttctcgaaaacccgtaacattcttcattccaaaacacatctggcttctcggaggtctggacaagtgattcttggcaacacatacctatagagacaataaaatcaaagtaataatggcaacacaatagataacatttaccaagcatacaccatgtggcagacacaattataagtgttttccatatttaacctacttaatcctcaggaataagccactgaggtcagtcctattattatccccatcttatagatgaagaaaatgaggcaccaggaagtcaaataacttgtcaaaggtcacaagactaggaaatacacaagtagaaatgtttacaattaaggcccaggctgggtttgccctcagttctgctatgcctcgcattatgccccaggaaactttttcccttgtgaaagccaagcttaaaaaaagaaaagccacatttgtaacgtgctctgttcccctgcctatggtgaggatcttcaaacagttatacatggacccagtccccctgccttctccttaatttcttaagtcatttgaaacagatggctgtcatggaaatagaatccagacatgttggtcagagttaaagatcaactaattccatcaaaaatagctcggcatgaaagggaactattctctggcttagtcatggatgagactttcaattgctataaagtggttcctttattagacaatgttaccagggaaacaacaggggtttgtttgacttctggggcccacaagtcaacaagagagccccatctaccaaggagcatgtccctgactacccctcagccagcagcaagacatggaccccagtcagggcaggagcagggtttcggcggcgcccagcacaagacattgcccctagagtctcagcccctaccctcgagtaatagatctgcctacctgagactgttgtttgcccaagagctgggtctcagcctgatgggaaccatataaaaaggttcactgacatactgcccacatgttgttctctttcattagatcttagcttccttgtctgctcttcattcttgcagtattcattcaacaaacattaaaaaaaaaaaaaagcattctatgtgtggaacactctgctagatgctgtggatttagaaatgaaaatacatcccgacccttggaatggaagggaaaggactgaagtaagacagattaagcaggaccgtcagcccagcttgaagcccagataaatacggagaacaagagagagcgagtagtgagagatgagtcccaatgcctcactttggtgacgggtgcgtggtgggcttcatgcagcttcttctgataaatgcctccttcagaactggtcaactctaccttggccagtgacccaggtggtcatagtagatttaccaagggaaaatggaaacttttattaggagctcttaggcctcttcacttcatggatttttttttcctttttttttgagatggagttttgccctgtcacccaggctggaatgcagtggtgcaatctcagctcactgcaacctccgcctcccaggttcaagcaattctcctgcctcagcctcccgagtagctgggactacaggtgtgcgccaccacaccaggctaatttttgtattttttgtaaagacaggttttcaccacgttggccaggctggtctgaactccagacctcaggtgattcacctgtctcagcctcccaaagtgctgggattacaggtgtgagccaccgtgcccggctacttcatggatttttgattacagattatgcctcttacaatttttaagaagaatcaagtgggctgaaggtcaatgtcaccataagacaaaagacatttttattagttgattctagggaattggccttaaggggagccctttcttcctaagagattcttaggtgattctcacttcctcttgccccagtattatttttgtttttggtatggctcactcagatccttttttcctcctatccctaagtaatccgggtttctttttcccatatttagaacaaaatgtatttatgcagagtgtgtccaaacctcaacccaaggcctgtatacaaaataaatcaaattaaacacatctttactgtcttctacctctttcctgacctcaatatatcccaacttgcctcactctgagaaccaaggctgtcccagcacctgagtcgcagatattctactgatttgacagaactgtgtgactatctggaacagcattttgatccacaatttgcccagttacaaagcttaaatgagctctagtgcatgcatatatatttcaaaattccaccatgatcttccacactctgtattgtaaatagagccctgtaatgcttttacttcgtatttcattgcttgttatacataaaaatatacttttcttcttcatgttagaaaatgcaaagaataggagggtgggggaatctctgggcttggagacaggagacttgccttcctactatggttccatcagaatgtagactgggacaatacaataattcaagtctggtttgctcatctgtaaattgggaagaatgtttccagctccagaatgctaaatctctaagtctgtggttggcagccactattgcagcagctcttcaatgactcaatgcagttttgcattctccctaccttttttttctaaaaccaataaaatagatacagcctttaggctttctgggatttcccttagtcaagctagggtcatcctgactttcggcgtgaatttgcaaaacaagacctgactctgtactcctgctctaaggactgtgcatggttccaaaggcttagcttgccagcatatttgagctttttccttctgttcaaactgttccaaaatataaaagaataaaattaattaagttggcactggacttccggtggtcagtcatgtgtgtcatctgtcacgtttttcgggctctggtggaaatggatctgtctgtcttctctcataggtggtattcacagccaacgactccggcccccgccgctacaccattgccgccctgctgagcccctactcctattccaccacggctgtcgtcaccaatcccaaggaatgagggacttctcctccagtggacctgaaggacgagggatgggatttcatgtaaccaagagtattccatttttactaaagcagtgttttcacctcatatgctatgttagaagtccaggcagagacaataaaacattcctgtgaaaggcacttttcattccactttaacttgattttttaaattcccttattgtcccttccaaaaaaaagagaatcaaaattttacaaagaatcaaaggaattctagaaagtatctgggcagaacgctaggagagatccaaatttccattgtcttgcaagcaaagcacgtattaaatatgatctgcagccattaaaaagacacattctgtaaatgagagagccttattttcctgtaaccttcagcaaatagcaaaagacacattccaagggcccacttctttactgtgggcactcgagataacttcgtataatgtatgctatacgaagttatatgcatgccagtagcagcacccacgtccaccttctgtctagtaatgtccaacacctccctcagtccaaacactgctctgcatccatgtggctcccatttatacctgaagcacttgatggggcctcaatgttttactagagcccacccccctgcaactctgagaccctctggatttgtctgtcagtgcctcactggggcgttggataatttcttaaaaggtcaagttccctcagcagcattctctgagcagtctgaagatgtgtgcttttcacagttcaaatccatgtggctgtttcacccacctgcctggccttgggttatctatcaggacctagcctagaagcaggtgtgtggcacttaacacctaagctgagtgactaactgaacactcaagtggatgccatctttgtcacttcttgactgtgacacaagcaactcctgatgccaaagccctgcccacccctctcatgcccatatttggacatggtacaggtcctcactggccatggtctgtgaggtcctggtcctctttgacttcataattcctaggggccactagtatctataagaggaagagggtgctggctcccaggccacagcccacaaaattccacctgctcacaggttggctggctcgacccaggtggtgtcccctgctctgagccagctcccggccaagccagcaccatgggaacccccaagaagaagaggaaggtgcgtaccgatttaaattccaatttactgaccgtacaccaaaatttgcctgcattaccggtcgatgcaacgagtgatgaggttcgcaagaacctgatggacatgttcagggatcgccaggcgttttctgagcatacctggaaaatgcttctgtccgtttgccggtcgtgggcggcatggtgcaagttgaataaccggaaatggtttcccgcagaacctgaagatgttcgcgattatcttctatatcttcaggcgcgcggtctggcagtaaaaactatccagcaacatttgggccagctaaacatgcttcatcgtcggtccgggctgccacgaccaagtgacagcaatgctgtttcactggttatgcggcggatccgaaaagaaaacgttgatgccggtgaacgtgcaaaacaggtaaatataaaatttttaagtgtataatgatgttaaactactgattctaattgtttgtgtattttaggctctagcgttcgaacgcactgatttcgaccaggttcgttcactcatggaaaatagcgatcgctgccaggatatacgtaatctggcatttctggggattgcttataacaccctgttacgtatagccgaaattgccaggatcagggttaaagatatctcacgtactgacggtgggagaatgttaatccatattggcagaacgaaaacgctggttagcaccgcaggtgtagagaaggcacttagcctgggggtaactaaactggtcgagcgatggatttccgtctctggtgtagctgatgatccgaataactacctgttttgccgggtcagaaaaaatggtgttgccgcgccatctgccaccagccagctatcaactcgcgccctggaagggatttttgaagcaactcatcgattgatttacggcgctaaggatgactctggtcagagatacctggcctggtctggacacagtgcccgtgtcggagccgcgcgagatatggcccgcgctggagtttcaataccggagatcatgcaagctggtggctggaccaatgtaaatattgtcatgaactatatccgtaacctggatagtgaaacaggggcaatggtgcgcctgctggaagatggcgattaggcggccggccgctaatcagccataccacatttgtagaggttttacttgctttaaaaaacctcccacacctccccctgaacctgaaacataaaatgaatgcaattgttgttgttaacttgtttattgcagcttataatggttacaaataaagcaatagcatcacaaatttcacaaataaagcatttttttcactgcattctagttgtggtttgtccaaactcatcaatgtatcttatcatgtctggatcccccggctagagtttaaacactagaactagtggatcccccgggatcatggcctccgcgccgggttttggcgcctcccgcgggcgcccccctcctcacggcgagcgctgccacgtcagacgaagggcgcagcgagcgtcctgatccttccgcccggacgctcaggacagcggcccgctgctcataagactcggccttagaaccccagtatcagcagaaggacattttaggacgggacttgggtgactctagggcactggttttctttccagagagcggaacaggcgaggaaaagtagtcccttctcggcgattctgcggagggatctccgtggggcggtgaacgccgatgattatataaggacgcgccgggtgtggcacagctagttccgtcgcagccgggatttgggtcgcggttcttgtttgtggatcgctgtgatcgtcacttggtgagtagcgggctgctgggctggccggggctttcgtggccgccgggccgctcggtgggacggaagcgtgtggagagaccgccaagggctgtagtctgggtccgcgagcaaggttgccctgaactgggggttggggggagcgcagcaaaatggcggctgttcccgagtcttgaatggaagacgcttgtgaggcgggctgtgaggtcgttgaaacaaggtggggggcatggtgggcggcaagaacccaaggtcttgaggccttcgctaatgcgggaaagctcttattcgggtgagatgggctggggcaccatctggggaccctgacgtgaagtttgtcactgactggagaactcggtttgtcgtctgttgcgggggcggcagttatggcggtgccgttgggcagtgcacccgtacctttgggagcgcgcgccctcgtcgtgtcgtgacgtcacccgttctgttggcttataatgcagggtggggccacctgccggtaggtgtgcggtaggcttttctccgtcgcaggacgcagggttcgggcctagggtaggctctcctgaatcgacaggcgccggacctctggtgaggggagggataagtgaggcgtcagtttctttggtcggttttatgtacctatcttcttaagtagctgaagctccggttttgaactatgcgctcggggttggcgagtgtgttttgtgaagttttttaggcaccttttgaaatgtaatcatttgggtcaatatgtaattttcagtgttagactagtaaattgtccgctaaattctggccgtttttggcttttttgttagacgtgttgacaattaatcatcggcatagtatatcggcatagtataatacgacaaggtgaggaactaaaccatgggatcggccattgaacaagatggattgcacgcaggttctccggccgcttgggtggagaggctattcggctatgactgggcacaacagacaatcggctgctctgatgccgccgtgttccggctgtcagcgcaggggcgcccggttctttttgtcaagaccgacctgtccggtgccctgaatgaactgcaggacgaggcagcgcggctatcgtggctggccacgacgggcgttccttgcgcagctgtgctcgacgttgtcactgaagcgggaagggactggctgctattgggcgaagtgccggggcaggatctcctgtcatctcaccttgctcctgccgagaaagtatccatcatggctgatgcaatgcggcggctgcatacgcttgatccggctacctgcccattcgaccaccaagcgaaacatcgcatcgagcgagcacgtactcggatggaagccggtcttgtcgatcaggatgatctggacgaagagcatcaggggctcgcgccagccgaactgttcgccaggctcaaggcgcgcatgcccgacggcgatgatctcgtcgtgacccatggcgatgcctgcttgccgaatatcatggtggaaaatggccgcttttctggattcatcgactgtggccggctgggtgtggcggaccgctatcaggacatagcgttggctacccgtgatattgctgaagagcttggcggcgaatgggctgaccgcttcctcgtgctttacggtatcgccgctcccgattcgcagcgcatcgccttctatcgccttcttgacgagttcttctgaggggatccgctgtaagtctgcagaaattgatgatctattaaacaataaagatgtccactaaaatggaagtttttcctgtcatactttgttaagaagggtgagaacagagtacctacattttgaatggaaggattggagctacgggggtgggggtggggtgggattagataaatgcctgctctttactgaaggctctttactattgctttatgataatgtttcatagttggatatcataatttaaacaagcaaaaccaaattaagggccagctcattcctcccactcatgatctatagatctatagatctctcgtgggatcattgtttttctcttgattcccactttgtggttctaagtactgtggtttccaaatgtgtcagtttcatagcctgaagaacgagatcagcagcctctgttccacatacacttcattctcagtattgttttgccaagttctaattccatcagacctcgacctgcagcccctagataacttcgtataatgtatgctatacgaagttatgctaggtaactataacggtcctaaggtagcgagctagcgagactcagcccaggaggaccaggatcttgccaaagcagtagcatcccatttgtaccaaaacagtgttcttgctctataaaccgtgttagcagctcagga

SEQ ID NO: 15 - DNA, 7476 bp, synthetic construct
  misc_feature 1..7476: note = Synthetic
  misc_feature 1..97: note = Mouse Sequence
  misc_feature 98..7298: note = Human Sequence
  misc_feature 7299..7376: note = Cassette LoxP Scar
  misc_feature 7377..7476: note = Mouse Sequence
  source 1..7476: mol_type = other DNA
agcttggcagggatcagcagcctgggttggaaggagggggtataaaagccccttcaccaggagaagccgtcacacagatccacaagctcctgacaggatggcttctcatcgtctgctcctcctctgccttgctggactggtatttgtgtctgaggctggccctacggtgagtgtttctgtgacatcccattcctacatttaagattcacgctaaatgaagtagaagtgactccttccagctttgccaaccagcttttattactagggcaagggtacccagcatctatttttaatataattaattcaaacttcaaaaagaatgaagttccactgagcttactgagctgggacttgaactctgagcattctacctcattgctttggtgcattaggtttgtaatatctggtacctctgtttcctcagatagatgatagaaataaagatatgatattaaggaagctgttaatactgaattttcagaaaagtatccctccataaaatgtatttgggggacaaactgcaggagattatattctggccctatagttattcaaaacgtatttattgattaatctttaaaaggcttagtgaacaatattctagtcagatatctaattcttaaatcctctagaagaattaactaatactataaaatgggtctggatgtagttctgacattattttataacaactggtaagagggagtgactatagcaacaactaaaatgatctcaggaaaacctgtttggccctatgtatggtacattacatcttttcagtaattccactcaaatggagacttttaacaaagcaactgttctcaggggacctattttctcccttaaaattcattatacacatccctggttgatagcagtgtgtctggaggcagaaaccattcttgctttggaaacaattacgtctgtgttatactgagtagggaagctcattaattgtcgacacttacgttcctgataatgggatcagtgtgtaattcttgtttcgctccagatttctaataccacaaagaataaatcctttcactctgatcaattttgttaacttctcacgtgtcttctctacacccagggcaccggtgaatccaagtgtcctctgatggtcaaagttctagatgctgtccgaggcagtcctgccatcaatgtggccgtgcatgtgttcagaaaggctgctgatgacacctgggagccatttgcctctgggtaagttgccaaagaaccctcccacaggacttggttttatcttcccgtttgcccctcacttggtagagagaggctcacatcatctgctaaagaatttacaagtagattgaaaaacgtaggcagaggtcaagtatgccctctgaaggatgccctctttttgttttgcttagctaggaagtgaccaggaacctgagcatcatttaggggcagacagtagagaaaagaaggaatcagaactcctctcctctagctgtggtttgcaacccttttgggtcacagaacactttatgtaggtgatgaaaagtaaacattctatgcccagaaaaaatgcacagatacacacacatacaaaatcatatatgtgattttaggagtttcacagattccctggtgtccctgggtaacaccaaagctaagtgtccttgtcttagaattttaggaaaaggtataatgtgtattaacccattaacaaaaggaaaggaattcagaaatattattaaccaggcatctgtctgtagttaatatggatcacccaaaacccaaggcttttgcctaatgaacactttggggcacctactgtgtgcaaggctgggggctgtcaagctcagttaaaaaaaaaaagatagaagagatggatccatgaggcaaagtacagccccaggctaatcccacgatcacccgacttcatgtccaagagtggcttctcaccttcattagccagttcacaattttcatggagtttttctacctgcactagcaaaaacttcaaggaaaatacatattaataaatctaagcaaagtgaccagaagacagagcaatcaggagaccctttgcatccagcagaagaggaactgctaagtatttacatctccacagagaagaatttctgttgggttttaattgaaccccaagaaccacatgattcttcaaccattattgggaagatcattttcttaggtctggttttaactggctttttatttgggaattcatttatgtttatataaaatgccaagcataacatgaaaagtggttacaggactattctaagggagagacagaatggacaccaaaaatattccaatgttcttgtgaatcttttccttgcaccaggacaaaaaaaaaaagaagtgaaaagaagaaaggaggaggggcataatcagagtcagtaaagacaactgctatttttatctatcgtagctgttgcagtcaaatgggaagcaatttccaacattcaactatggagctggtacttacatggaaatagaagttgcctagtgtttgttgctggcaaagagttatcagagaggttaaatatataaaagggaaaagagtcagatacaggttcttcttcctactttaggttttccactgtgtgtgcaaatgatactccctggtggtgtgcagatgcctcaaagctatcctcacaccacaagggagaggagcgagatcctgctgtcctggagaagtgcagagttagaacagctgtggccacttgcatccaatcatcaatcttgaatcacagggactctttcttaagtaaacattatacctggccgggcacggtggctcacgcctgtaatcccagcactttgggatgccaaagtgggcatatcatctgaggtcaggagttcaagaccagcctggccaacatggcaaaactccgtctttatgaaaaatacaaaaattagccaggcatggtggcaggcgcctgtaatcccagctaattgggaggctgaggctggagaatcccttgaatctaggaggcagaggttgcagtgagctgagatcgtgccattgcactccagcctgggtgacaagagtaaaactctgtctcaaaaaaaaaaaattatacctacattctcttcttatcagagaaaaaaatctacagtgagcttttcaaaaagtttttacaaactttttgccatttaatttcagttaggagttttccctacttctgacttagttgaggggaaatgttcataacatgtttataacatgtttatgtgtgttagttggtgggggtgtattactttgccatgccatttgtttcctccatgcgtaacttaatccagactttcacaccttataggaaaaccagtgagtctggagagctgcatgggctcacaactgaggaggaatttgtagaagggatatacaaagtggaaatagacaccaaatcttactggaaggcacttggcatctccccattccatgagcatgcagaggtgagtatacagaccttcgagggttgttttggttttggtttttgcttttggcattccaggaaatgcacagttttactcagtgtaccacagaaatgtcctaaggaaggtgatgaatgaccaaaggttccctttcctattatacaagaaaaaattcacaacactctgagaagcaaatttctttttgactttgatgaaaatccacttagtaacatgacttgaacttacatgaaactactcatagtctattcattccactttatatgaatattgatgtatctgctgttgaaataatagtttatgaggcagccctccagaccccacgtagagtgtatgtaacaagagatgcaccattttatttctcgaaaacccgtaacattcttcattccaaaacacatctggcttctcggaggtctggacaagtgattcttggcaacacatacctatagagacaataaaatcaaagtaataatggcaacacaatagataacatttaccaagcatacaccatgtggcagacacaattataagtgttttccatatttaacctacttaatcctcaggaataagccactgaggtcagtcctattattatccccatcttatagatgaagaaaatgaggcaccaggaagtcaaataacttgtcaaaggtcacaagactaggaaatacacaagtagaaatgtttacaattaaggcccaggctgggtttgccctcagttctgctatgcctcgcattatgccccaggaaactttttcccttgtgaaagccaagcttaaaaaaagaaaagccacatttgtaacgtgctctgttcccctgcctatggtgaggatcttcaaacagttatacatggacccagtccccctgccttctccttaatttcttaagtcatttgaaacagatggctgtcatggaaatagaatccagacatgttggtcagagttaaagatcaactaattccatcaaaaatagctcggcatgaaagggaactattctctggcttagtcatggatgagactttcaattgctataaagtggttcctttattagacaatgttaccagggaaacaacaggggtttgtttgacttctggggcccacaagtcaacaagagagccccatctaccaaggagcatgtccctgactacccctcagccagcagcaagacatggaccccagtcagggcaggagcagggtttcggcggcgcccagcacaagacattgcccctagagtctcagcccctaccctcgagtaatagatctgcctacctgagactgttgtttgcccaagagctgggtctcagcctgatgggaaccatataaaaaggttcactgacatactgcccacatgttgttctctttcattagatcttagcttccttgtctgctcttcattcttgcagtattcattcaacaaacattaaaaaaaaaaaaaagcattctatgtgtggaacactctgctagatgctgtggatttagaaatgaaaatacatcccgacccttggaatggaagggaaaggactgaagtaagacagattaagcaggaccgtcagcccagcttgaagcccagataaatacggagaacaagagagagcgagtagtgagagatgagtcccaatgcctcactttggtgacgggtgcgtggtgggcttcatgcagcttcttctgataaatgcctccttcagaactggtcaactctaccttggccagtgacccaggtggtcatagtagatttaccaagggaaaatggaaacttttattaggagctcttaggcctcttcacttcatggatttttttttcctttttttttgagatggagttttgccctgtcacccaggctggaatgcagtggtgcaatctcagctcactgcaacctccgcctcccaggttcaagcaattctcctgcctcagcctcccgagtagctgggactacaggtgtgcgccaccacaccaggctaatttttgtattttttgtaaagacaggttttcaccacgttggccaggctggtctgaactccagacctcaggtgattcacctgtctcagcctcccaaagtgctgggattacaggtgtgagccaccgtgcccggctacttcatggatttttgattacagattatgcctcttacaatttttaagaagaatcaagtgggctgaaggtcaatgtcaccataagacaaaagacatttttattagttgattctagggaattggccttaaggggagccctttcttcctaagagattcttaggtgattctcacttcctcttgccccagtattatttttgtttttggtatggctcactcagatccttttttcctcctatccctaagtaatccgggtttctttttcccatatttagaacaaaatgtatttatgcagagtgtgtccaaacctcaacccaaggcctgtatacaaaataaatcaaattaaacacatctttactgtcttctacctctttcctgacctcaatatatcccaacttgcctcactctgagaaccaaggctgtcccagcacctgagtcgcagatattctactgatttgacagaactgtgtgactatctggaacagcattttgatccacaatttgcccagttacaaagcttaaatgagctctagtgcatgcatatatatttcaaaattccaccatgatcttccacactctgtattgtaaatagagccctgtaatgcttttacttcgtatttcattgcttgttatacataaaaatatacttttcttcttcatgttagaaaatgcaaagaataggagggtgggggaatctctgggcttggagacaggagacttgccttcctactatggttccatcagaatgtagactgggacaatacaataattcaagtctggtttgctcatctgtaaattgggaagaatgtttccagctccagaatgctaaatctctaagtctgtggttggcagccactattgcagcagctcttcaatgactcaatgcagttttgcattctccctaccttttttttctaaaaccaataaaatagatacagcctttaggctttctgggatttcccttagtcaagctagggtcatcctgactttcggcgtgaatttgcaaaacaagacctgactctgtactcctgctctaaggactgtgcatggttccaaaggcttagcttgccagcatatttgagctttttccttctgttcaaactgttccaaaatataaaagaataaaattaattaagttggcactggacttccggtggtcagtcatgtgtgtcatctgtcacgtttttcgggctctggtggaaatggatctgtctgtcttctctcataggtggtattcacagccaacgactccggcccccgccgctacaccattgccgccctgctgagcccctactcctattccaccacggctgtcgtcaccaatcccaaggaatgagggacttctcctccagtggacctgaaggacgagggatgggatttcatgtaaccaagagtattccatttttactaaagcagtgttttcacctcatatgctatgttagaagtccaggcagagacaataaaacattcctgtgaaaggcacttttcattccactttaacttgattttttaaattcccttattgtcccttccaaaaaaaagagaatcaaaattttacaaagaatcaaaggaattctagaaagtatctgggcagaacgctaggagagatccaaatttccattgtcttgcaagcaaagcacgtattaaatatgatctgcagccattaaaaagacacattctgtaaatgagagagccttattttcctgtaaccttcagcaaatagcaaaagacacattccaagggcccacttctttactgtgggcactcgagataacttcgtataatgtatgctatacgaagttatgctaggtaactataacggtcctaaggtagcgagctagcgagactcagcccaggaggaccaggatcttgccaaagcagtagcatcccatttgtaccaaaacagtgttcttgctctataaaccgtgttagcagctcagga

SEQ ID NO: 16 - DNA, 11218 bp, synthetic construct
  misc_feature 1..11218: note = Synthetic
  misc_feature 1..100: note = Mouse Sequence
  misc_feature 101..6308: note = Human Sequence
  misc_feature 6309..11118: note = SDC Neo Cassette
  misc_feature 11119..11218: note = Mouse Sequence
  source 1..11218: mol_type = other DNA
atgtacttttggttttgttccagagtctatcaccggaaagaacaagccggtttactctgacccatttcactgacatttctcttgtctcctctgtgcccagggcaccggtgaatccaagtgtcctctgatggtcaaagttctagatgctgtccgaggcagtcctgccatcaatgtggccgtgcatgtgttcagaaaggctgctgatgacacctgggagccatttgcctctgggtaagttgccaaagaaccctcccacaggacttggttttatcttcccgtttgcccctcacttggtagagagaggctcacatcatctgctaaagaatttacaagtagattgaaaaacgtaggcagaggtcaagtatgccctctgaaggatgccctctttttgttttgcttagctaggaagtgaccaggaacctgagcatcatttaggggcagacagtagagaaaagaaggaatcagaactcctctcctctagctgtggtttgcaacccttttgggtcacagaacactttatgtaggtgatgaaaagtaaacattctatgcccagaaaaaatgcacagatacacacacatacaaaatcatatatgtgattttaggagtttcacagattccctggtgtccctgggtaacaccaaagctaagtgtccttgtcttagaattttaggaaaaggtataatgtgtattaacccattaacaaaaggaaaggaattcagaaatattattaaccaggcatctgtctgtagttaatatggatcacccaaaacccaaggcttttgcctaatgaacactttggggcacctactgtgtgcaaggctgggggctgtcaagctcagttaaaaaaaaaaagatagaagagatggatccatgaggcaaagtacagccccaggctaatcccacgatcacccgacttcatgtccaagagtggcttctcaccttcattagccagttcacaattttcatggagtttttctacctgcactagcaaaaacttcaaggaaaatacatattaataaatctaagcaaagtgaccagaagacagagcaatcaggagaccctttgcatccagcagaagaggaactgctaagtatttacatctccacagagaagaatttctgttgggttttaattgaaccccaagaaccacatgattcttcaaccattattgggaagatcattttcttaggtctggttttaactggctttttatttgggaattcatttatgtttatataaaatgccaagcataacatgaaaagtggttacaggactattctaagggagagacagaatggacaccaaaaatattccaatgttcttgtgaatcttttccttgcaccaggacaaaaaaaaaaagaagtgaaaagaagaaaggaggaggggcataatcagagtcagtaaagacaactgctatttttatctatcgtagctgttgcagtcaaatgggaagcaatttccaacattcaactatggagctggtacttacatggaaatagaagttgcctagtgtttgttgctggcaaagagttatcagagaggttaaatatataaaagggaaaagagtcagatacaggttcttcttcctactttaggttttccactgtgtgtgcaaatgatactccctggtggtgtgcagatgcctcaaagctatcctcacaccacaagggagaggagcgagatcctgctgtcctggagaagtgcagagttagaacagctgtggccacttgcatccaatcatcaatcttgaatcacagggactctttcttaagtaaacattatacctggccgggcacggtggctcacgcctgtaatcccagcactttgggatgccaaagtgggcatatcatctgaggtcaggagttcaagaccagcctggccaacatggcaaaactccgtctttatgaaaaatacaaaaattagccaggcatggtggcaggcgcctgtaatcccagctaattgggaggctgaggctggagaatcccttgaatctaggaggcagaggttgcagtgagctgagatcgtgccattgcactccagcctgggtgacaagagtaaaactctgtctcaaaaaaaaaaaattatacctacattctcttcttatcagagaaaaaaatctacagtgagcttttcaaaaagtttttacaaactttttgccatttaatttcagttaggagttttccctacttctgacttagttgaggggaaatgttcataacatgtttataacatgtttatgtgtgttagttggtgggggtgtattactttgccatgccatttgtttcctccatgcgtaacttaatccagactttcacaccttataggaaaaccagtgagtctggagagctgcatgggctcacaactgaggaggaatttgtagaagggatatacaaagtggaaatagacaccaaatcttactggaaggcacttggcatctccccattccatgagcatgcagaggtgagtatacagaccttcgagggttgttttggttttggtttttgcttttggcattccaggaaatgcacagttttactcagtgtaccacagaaatgtcctaaggaaggtgatgaatgaccaaaggttccctttcctattatacaagaaaaaattcacaacactctgagaagcaaatttctttttgactttgatgaaaatccacttagtaacatgacttgaacttacatgaaactactcatagtctattcattccactttatatgaatattgatgtatctgctgttgaaataatagtttatgaggcagccctccagaccccacgtagagtgtatgtaacaagagatgcaccattttatttctcgaaaacccgtaacattcttcattccaaaacacatctggcttctcggaggtctggacaagtgattcttggcaacacatacctatagagacaataaaatcaaagtaataatggcaacacaatagataacatttaccaagcatacaccatgtggcagacacaattataagtgttttccatatttaacctacttaatcctcaggaataagccactgaggtcagtcctattattatccccatcttatagatgaagaaaatgaggcaccaggaagtcaaataacttgtcaaaggtcacaagactaggaaatacacaagtagaaatgtttacaattaaggcccaggctgggtttgccctcagttctgctatgcctcgcattatgccccaggaaactttttcccttgtgaaagccaagcttaaaaaaagaaaagccacatttgtaacgtgctctgttcccctgcctatggtgaggatcttcaaacagttatacatggacccagtccccctgccttctccttaatttcttaagtcatttgaaacagatggctgtcatggaaatagaatccagacatgttggtcagagttaaagatcaactaattccatcaaaaatagctcggcatgaaagggaactattctctggcttagtcatggatgagactttcaattgctataaagtggttcctttattagacaatgttaccagggaaacaacaggggtttgtttgacttctggggcccacaagtcaacaagagagccccatctaccaaggagcatgtccctgactacccctcagccagcagcaagacatggaccccagtcagggcaggagcagggtttcggcggcgcccagcacaagacattgcccctagagtctcagcccctaccctcgagtaatagatctgcctacctgagactgttgtttgcccaagagctgggtctcagcctgatgggaaccatataaaaaggttcactgacatactgcccacatgttgttctctttcattagatcttagcttccttgtctgctcttcattcttgcagtattcattcaacaaacattaaaaaaaaaaaaaagcattctatgtgtggaacactctgctagatgctgtggatttagaaatgaaaatacatcccgacccttggaatggaagggaaaggactgaagtaagacagattaagcaggaccgtcagcccagcttgaagcccagataaatacggagaacaagagagagcgagtagtgagagatgagtcccaatgcctcactttggtgacgggtgcgtggtgggcttcatgcagcttcttctgataaatgcctccttcagaactggtcaactctaccttggccagtgacccaggtggtcatagtagatttaccaagggaaaatggaaacttttattaggagctcttaggcctcttcacttcatggatttttttttcctttttttttgagatggagttttgccctgtcacccaggctggaatgcagtggtgcaatctcagctcactgcaacctccgcctcccaggttcaagcaattctcctgcctcagcctcccgagtagctgggactacaggtgtgcgccaccacaccaggctaatttttgtattttttgtaaagacaggttttcaccacgttggccaggctggtctgaactccagacctcaggtgattcacctgtctcagcctcccaaagtgctgggattacaggtgtgagccaccgtgcccggctacttcatggatttttgattacagattatgcctcttacaatttttaagaagaatcaagtgggctgaaggtcaatgtcaccataagacaaaagacatttttattagttgattctagggaattggccttaaggggagccctttcttcctaagagattcttaggtgattctcacttcctcttgccccagtattatttttgtttttggtatggctcactcagatccttttttcctcctatccctaagtaatccgggtttctttttcccatatttagaacaaaatgtatttatgcagagtgtgtccaaacctcaacccaaggcctgtatacaaaataaatcaaattaaacacatctttactgtcttctacctctttcctgacctcaatatatcccaacttgcctcactctgagaaccaaggctgtcccagcacctgagtcgcagatattctactgatttgacagaactgtgtgactatctggaacagcattttgatccacaatttgcccagttacaaagcttaaatgagctctagtgcatgcatatatatttcaaaattccaccatgatcttccacactctgtattgtaaatagagccctgtaatgcttttacttcgtatttcattgcttgttatacataaaaatatacttttcttcttcatgttagaaaatgcaaagaataggagggtgggggaatctctgggcttggagacaggagacttgccttcctactatggttccatcagaatgtagactgggacaatacaataattcaagtctggtttgctcatctgtaaattgggaagaatgtttccagctccagaatgctaaatctctaagtctgtggttggcagccactattgcagcagctcttcaatgactcaatgcagttttgcattctccctaccttttttttctaaaaccaataaaatagatacagcctttaggctttctgggatttcccttagtcaagctagggtcatcctgactttcggcgtgaatttgcaaaacaagacctgactctgtactcctgctctaaggactgtgcatggttccaaaggcttagcttgccagcatatttgagctttttccttctgttcaaactgttccaaaatataaaagaataaaattaattaagttggcactggacttccggtggtcagtcatgtgtgtcatctgtcacgtttttcgggctctggtggaaatggatctgtctgtcttctctcataggtggtattcacagccaacgactccggcccccgccgctacaccattgccgccctgctgagcccctactcctattccaccacggctgtcgtcaccaatcccaaggaatgagggacttctcctccagtggacctgaaggacgagggatgggatttcatgtaaccaagagtattccatttttactaaagcagtgttttcacctcatatgctatgttagaagtccaggcagagacaataaaacattcctgtgaaaggcacttttcattccactttaacttgattttttaaattcccttattgtcccttccaaaaaaaagagaatcaaaattttacaaagaatcaaaggaattctagaaagtatctgggcagaacgctaggagagatccaaatttccattgtcttgcaagcaaagcacgtattaaatatgatctgcagccattaaaaagacacattctgtaaatgagagagccttattttcctgtaaccttcagcaaatagcaaaagacacattccaagggcccacttctttactgtgggcactcgagataacttcgtataatgtatgctatacgaagttatatgcatgccagtagcagcacccacgtccaccttctgtctagtaatgtccaacacctccctcagtccaaacactgctctgcatccatgtggctcccatttatacctgaagcacttgatggggcctcaatgttttactagagcccacccccctgcaactctgagaccctctggatttgtctgtcagtgcctcactggggcgttggataatttcttaaaaggtcaagttccctcagcagcattctctgagcagtctgaagatgtgtgcttttcacagttcaaatccatgtggctgtttcacccacctgcctggccttgggttatctatcaggacctagcctagaagcaggtgtgtggcacttaacacctaagctgagtgactaactgaacactcaagtggatgccatctttgtcacttcttgactgtgacacaagcaactcctgatgccaaagccctgcccacccctctcatgcccatatttggacatggtacaggtcctcactggccatggtctgtgaggtcctggtcctctttgacttcataattcctaggggccactagtatctataagaggaagagggtgctggctcccaggccacagcccacaaaattccacctgctcacaggttggctggctcgacccaggtggtgtcccctgctctgagccagctcccggccaagccagcaccatgggaacccccaagaagaagaggaaggtgcgtaccgatttaaattccaatttactgaccgtacaccaaaatttgcctgcattaccggtcgatgcaacgagtgatgaggttcgcaagaacctgatggacatgttcagggatcgccaggcgttttctgagcatacctggaaaatgcttctgtccgtttgccggtcgtgggcggcatggtgcaagttgaataaccggaaatggtttcccgcagaacctgaagatgttcgcgattatcttctatatcttcaggcgcgcggtctggcagtaaaaactatccagcaacatttgggccagctaaacatgcttcatcgtcggtccgggctgccacgaccaagtgacagcaatgctgtttcactggttatgcggcggatccgaaaagaaaacgttgatgccggtgaacgtgcaaaacaggtaaatataaaatttttaagtgtataatgatgttaaactactgattctaattgtttgtgtattttaggctctagcgttcgaacgcactgatttcgaccaggttcgttcactcatggaaaatagcgatcgctgccaggatatacgtaatctggcatttctggggattgcttataacaccctgttacgtatagccgaaattgccaggatcagggttaaagatatctcacgtactgacggtgggagaatgttaatccatattggcagaacgaaaacgctggttagcaccgcaggtgtagagaaggcacttagcctgggggtaactaaactggtcgagcgatggatttccgtctctggtgtagctgatgatccgaataactacctgttttgccgggtcagaaaaaatggtgttgccgcgccatctgccaccagccagctatcaactcgcgccctggaagggatttttgaagcaactcatcgattgatttacggcgctaaggatgactctggtcagagatacctggcctggtctggacacagtgcccgtgtcggagccgcgcgagatatggcccgcgctggagtttcaataccggagatcatgcaagctggtggctggaccaatgtaaatattgtcatgaactatatccgtaacctggatagtgaaacaggggcaatggtgcgcctgctggaagatggcgattaggcggccggccgctaatcagccataccacatttgtagaggttttacttgctttaaaaaacctcccacacctccccctgaacctgaaacataaaatgaatgcaattgttgttgttaacttgtttattgcagcttataatggttacaaataaagcaatagcatcacaaatttcacaaataaagcatttttttcactgcattctagttgtggtttgtccaaactcatcaatgtatcttatcatgtctggatcccccggctagagtttaaacactagaactagtggatcccccgggatcatggcctccgcgccgggttttggcgcctcccgcgggcgcccccctcctcacggcgagcgctgccacgtcagacgaagggcgcagcgagcgtcctgatccttccgcccggacgctcaggacagcggcccgctgctcataagactcggccttagaaccccagtatcagcagaaggacattttaggacgggacttgggtgactctagggcactggttttctttccagagagcggaacaggcgaggaaaagtagtcccttctcggcgattctgcggagggatctccgtggggcggtgaacgccgatgattatataaggacgcgccgggtgtggcacagctagttccgtcgcagccgggatttgggtcgcggttcttgtttgtggatcgctgtgatcgtcacttggtgagtagcgggctgctgggctggccggggctttcgtggccgccgggccgctcggtgggacggaagcgtgtggagagaccgccaagggctgtagtctgggtccgcgagcaaggttgccctgaactgggggttggggggagcgcagcaaaatggcggctgttcccgagtcttgaatggaagacgcttgtgaggcgggctgtgaggtcgttgaaacaaggtggggggcatggtgggcggcaagaacccaaggtcttgaggccttcgctaatgcgggaaagctcttattcgggtgagatgggctggggcaccatctggggaccctgacgtgaagtttgtcactgactggagaactcggtttgtcgtctgttgcgggggcggcagttatggcggtgccgttgggcagtgcacccgtacctttgggagcgcgcgccctcgtcgtgtcgtgacgtcacccgttctgttggcttataatgcagggtggggccacctgccggtaggtgtgcggtaggcttttctccgtcgcaggacgcagggttcgggcctagggtaggctctcctgaatcgacaggcgccggacctctggtgaggggagggataagtgaggcgtcagtttctttggtcggttttatgtacctatcttcttaagtagctgaagctccggttttgaactatgcgctcggggttggcgagtgtgttttgtgaagttttttaggcaccttttgaaatgtaatcatttgggtcaatatgtaattttcagtgttagactagtaaattgtccgctaaattctggccgtttttggcttttttgttagacgtgttgacaattaatcatcggcatagtatatcggcatagtataatacgacaaggtgaggaactaaaccatgggatcggccattgaacaagatggattgcacgcaggttctccggccgcttgggtggagaggctattcggctatgactgggcacaacagacaatcggctgctctgatgccgccgtgttccggctgtcagcgcaggggcgcccggttctttttgtcaagaccgacctgtccggtgccctgaatgaactgcaggacgaggcagcgcggctatcgtggctggccacgacgggcgttccttgcgcagctgtgctcgacgttgtcactgaagcgggaagggactggctgctattgggcgaagtgccggggcaggatctcctgtcatctcaccttgctcctgccgagaaagtatccatcatggctgatgcaatgcggcggctgcatacgcttgatccggctacctgcccattcgaccaccaagcgaaacatcgcatcgagcgagcacgtactcggatggaagccggtcttgtcgatcaggatgatctggacgaagagcatcaggggctcgcgccagccgaactgttcgccaggctcaaggcgcgcatgcccgacggcgatgatctcgtcgtgacccatggcgatgcctgcttgccgaatatcatggtggaaaatggccgcttttctggattcatcgactgtggccggctgggtgtggcggaccgctatcaggacatagcgttggctacccgtgatattgctgaagagcttggcggcgaatgggctgaccgcttcctcgtgctttacggtatcgccgctcccgattcgcagcgcatcgccttctatcgccttcttgacgagttcttctgaggggatccgctgtaagtctgcagaaattgatgatctattaaacaataaagatgtccactaaaatggaagtttttcctgtcatactttgttaagaagggtgagaacagagtacctacattttgaatggaaggattggagctacgggggtgggggtggggtgggattagataaatgcctgctctttactgaaggctctttactattgctttatgataatgtttcatagttggatatcataatttaaacaagcaaaaccaaattaagggccagctcattcctcccactcatgatctatagatctatagatctctcgtgggatcattgtttttctcttgattcccactttgtggttctaagtactgtggtttccaaatgtgtcagtttcatagcctgaagaacgagatcagcagcctctgttccacatacacttcattctcagtattgttttgccaagttctaattccatcagacctcgacctgcagcccctagataacttcgtataatgtatgctatacgaagttatgctaggtaactataacggtcctaaggtagcgagctagcgagactcagcccaggaggaccaggatcttgccaaagcagtagcatcccatttgtaccaaaacagtgttcttgctctataaaccgtgttagcagctcagga

SEQ ID NO: 17 - DNA, 6486 bp, synthetic construct
  misc_feature 1..6486: note = Synthetic
  misc_feature 1..100: note = Mouse Sequence
  misc_feature 101..6308: note = Human Sequence
  misc_feature 6309..6386: note = Cassette LoxP Scar
  misc_feature 6387..6486: note = Mouse Sequence
  source 1..6486: mol_type = other DNA
atgtacttttggttttgttccagagtctatcaccggaaagaacaagccggtttactctgacccatttcactgacatttctcttgtctcctctgtgcccagggcaccggtgaatccaagtgtcctctgatggtcaaagttctagatgctgtccgaggcagtcctgccatcaatgtggccgtgcatgtgttcagaaaggctgctgatgacacctgggagccatttgcctctgggtaagttgccaaagaaccctcccacaggacttggttttatcttcccgtttgcccctcacttggtagagagaggctcacatcatctgctaaagaatttacaagtagattgaaaaacgtaggcagaggtcaagtatgccctctgaaggatgccctctttttgttttgcttagctaggaagtgaccaggaacctgagcatcatttaggggcagacagtagagaaaagaaggaatcagaactcctctcctctagctgtggtttgcaacccttttgggtcacagaacactttatgtaggtgatgaaaagtaaacattctatgcccagaaaaaatgcacagatacacacacatacaaaatcatatatgtgattttaggagtttcacagattccctggtgtccctgggtaacaccaaagctaagtgtccttgtcttagaattttaggaaaaggtataatgtgtattaacccattaacaaaaggaaaggaattcagaaatattattaaccaggcatctgtctgtagttaatatggatcacccaaaacccaaggcttttgcctaatgaacactttggggcacctactgtgtgcaaggctgggggctgtcaagctcagttaaaaaaaaaaagatagaagagatggatccatgaggcaaagtacagccccaggctaatcccacgatcacccgacttcatgtccaagagtggcttctcaccttcattagccagttcacaattttcatggagtttttctacctgcactagcaaaaacttcaaggaaaatacatattaataaatctaagcaaagtgaccagaagacagagcaatcaggagaccctttgcatccagcagaagaggaactgctaagtatttacatctccacagagaagaatttctgttgggttttaattgaaccccaagaaccacatgattcttcaaccattattgggaagatcattttcttaggtctggttttaactggctttttatttgggaattcatttatgtttatataaaatgccaagcataacatgaaaagtggttacaggactattctaagggagagacagaatggacaccaaaaatattccaatgttcttgtgaatcttttccttgcaccaggacaaaaaaaaaaagaagtgaaaagaagaaaggaggaggggcataatcagagtcagtaaagacaactgctatttttatctatcgtagctgttgcagtcaaatgggaagcaatttccaacattcaactatggagctggtacttacatggaaatagaagttgcctagtgtttgttgctggcaaagagttatcagagaggttaaatatataaaagggaaaagagtcagatacaggttcttcttcctactttaggttttccactgtgtgtgcaaatgatactccctggtggtgtgcagatgcctcaaagctatcctcacaccacaagggagaggagcgagatcctgctgtcctggagaagtgcagagttagaacagctgtggccacttgcatccaatcatcaatcttgaatcacagggactctttcttaagtaaacattatacctggccgggcacggtggctcacgcctgtaatcccagcactttgggatgccaaagtgggcatatcatctgaggtcaggagttcaagaccagcctggccaacatggcaaaactccgtctttatgaaaaatacaaaaattagccaggcatggtggcaggcgcctgtaatcccagctaattgggaggctgaggctggagaatcccttgaatctaggaggcagaggttgcagtgagctgagatcgtgccattgcactccagcctgggtgacaagagtaaaactctgtctcaaaaaaaaaaaattatacctacattctcttcttatcagagaaaaaaatctacagtgagcttttcaaaaagtttttacaaactttttgccatttaatttcagttaggagttttccctacttctgacttagttgaggggaaatgttcataacatgtttataacatgtttatgtgtgttagttggtgggggtgtattactttgccatgccatttgtttcctccatgcgtaacttaatccagactttcacaccttataggaaaaccagtgagtctggagagctgcatgggctcacaactgaggaggaatttgtagaagggatatacaaagtggaaatagacaccaaatcttactggaaggcacttggcatctccccattccatgagcatgcagaggtgagtatacagaccttcgagggttgttttggttttggtttttgcttttggcattccaggaaatgcacagttttactcagtgtaccacagaaatgtcctaaggaaggtgatgaatgaccaaaggttccctttcctattatacaagaaaaaattcacaacactctgagaagcaaatttctttttgactttgatgaaaatccacttagtaacatgacttgaacttacatgaaactactcatagtctattcattccactttatatgaatattgatgtatctgctgttgaaataatagtttatgaggcagccctccagaccccacgtagagtgtatgtaacaagagatgcaccattttatttctcgaaaacccgtaacattcttcattccaaaacacatctggcttctcggaggtctggacaagtgattcttggcaacacatacctatagagacaataaaatcaaagtaataatggcaacacaatagataacatttaccaagcatacaccatgtggcagacacaattataagtgttttccatatttaacctacttaatcctcaggaataagccactgaggtcagtcctattattatccccatcttatagatgaagaaaatgaggcaccaggaagtcaaataacttgtcaaaggtcacaagactaggaaatacacaagtagaaatgtttacaattaaggcccaggctgggtttgccctcagttctgctatgcctcgcattatgccccaggaaactttttcccttgtgaaagccaagcttaaaaaaagaaaagccacatttgtaacgtgctctgttcccctgcctatggtgaggatcttcaaacagttatacatggacccagtccccctgccttctccttaatttcttaagtcatttgaaacagatggctgtcatggaaatagaatccagacatgttggtcagagttaaagatcaactaattccatcaaaaatagctcggcatgaaagggaactattctctggcttagtcatggatgagactttcaattgctataaagtggttcctttattagacaatgttaccagggaaacaacaggggtttgtttgacttctggggcccacaagtcaacaagagagccccatctaccaaggagcatgtccctgactacccctcagccagcagcaagacatggaccccagtcagggcaggagcagggtttcggcggcgcccagcacaagacattgcccctagagtctcagcccctaccctcgagtaatagatctgcctacctgagactgttgtttgcccaagagctgggtctcagcctgatgggaaccatataaaaaggttcactgacatactgcccacatgttgttctctttcattagatcttagcttccttgtctgctcttcattcttgcagtattcattcaacaaacattaaaaaaaaaaaaaagcattctatgtgtggaacactctgctagatgctgtggatttagaaatgaaaatacatcccgacccttggaatggaagggaaaggactgaagtaagacagattaagcaggaccgtcagcccagcttgaagcccagataaatacggagaacaagagagagcgagtagtgagagatgagtcccaatgcctcactttggtgacgggtgcgtggtgggcttcatgcagcttcttctgataaatgcctccttcagaactggtcaactctaccttggccagtgacccaggtggtcatagtagatttaccaagggaaaatggaaacttttattaggagctcttaggcctcttcacttcatggatttttttttcctttttttttgagatggagttttgccctgtcacccaggctggaatgcagtggtgcaatctcagctcactgcaacctccgcctcccaggttcaagcaattctcctgcctcagcctcccgagtagctgggactacaggtgtgcgccaccacaccaggctaatttttgtattttttgtaaagacaggttttcaccacgttggccaggctggtctgaactccagacctcaggtgattcacctgtctcagcctcccaaagtgctgggattacaggtgtgagccaccgtgcccggctacttcatggatttttgattacagattatgcctcttacaatttttaagaagaatcaagtgggctgaaggtcaatgtcaccataagacaaaagacatttttattagttgattctagggaattggccttaaggggagccctttcttcctaagagattcttaggtgattctcacttcctcttgccccagtattatttttgtttttggtatggctcactcagatccttttttcctcctatccctaagtaatccgggtttctttttcccatatttagaacaaaatgtatttatgcagagtgtgtccaaacctcaacccaaggcctgtatacaaaataaatcaaattaaacacatctttactgtcttctacctctttcctgacctcaatatatcccaacttgcctcactctgagaaccaaggctgtcccagcacctgagtcgcagatattctactgatttgacagaactgtgtgactatctggaacagcattttgatccacaatttgcccagttacaaagcttaaatgagctctagtgcatgcatatatatttcaaaattccaccatgatcttccacactctgtattgtaaatagagccctgtaatgcttttacttcgtatttcattgcttgttatacataaaaatatacttttcttcttcatgttagaaaatgcaaagaataggagggtgggggaatctctgggcttggagacaggagacttgccttcctactatggttccatcagaatgtagactgggacaatacaataattcaagtctggtttgctcatctgtaaattgggaagaatgtttccagctccagaatgctaaatctctaagtctgtggttggcagccactattgcagcagctcttcaatgactcaatgcagttttgcattctccctaccttttttttctaaaaccaataaaatagatacagcctttaggctttctgggatttcccttagtcaagctagggtcatcctgactttcggcgtgaatttgcaaaacaagacctgactctgtactcctgctctaaggactgtgcatggttccaaaggcttagcttgccagcatatttgagctttttccttctgttcaaactgttccaaaatataaaagaataaaattaattaagttggcactggacttccggtggtcagtcatgtgtgtcatctgtcacgtttttcgggctctggtggaaatggatctgtctgtcttctctcataggtggtattcacagccaacgactccggcccccgccgctacaccattgccgccctgctgagcccctactcctattccaccacggctgtcgtcaccaatcccaaggaatgagggacttctcctccagtggacctgaaggacgagggatgggatttcatgtaaccaagagtattccatttttactaaagcagtgttttcacctcatatgctatgttagaagtccaggcagagacaataaaacattcctgtgaaaggcacttttcattccactttaacttgattttttaaattcccttattgtcccttccaaaaaaaagagaatcaaaattttacaaagaatcaaaggaattctagaaagtatctgggcagaacgctaggagagatccaaatttccattgtcttgcaagcaaagcacgtattaaatatgatctgcagccattaaaaagacacattctgtaaatgagagagccttattttcctgtaaccttcagcaaatagcaaaagacacattccaagggcccacttctttactgtgggcactcgagataacttcgtataatgtatgctatacgaagttatgctaggtaactataacggtcctaaggtagcgagctagcgagactcagcccaggaggaccaggatcttgccaaagcagtagcatcccatttgtaccaaaacagtgttcttgctctataaaccgtgttagcagctcagga

SEQ ID NO: 18 - DNA, 7201 bp, Homo sapiens
  source 1..7201: mol_type = other DNA
atggcttctcatcgtctgctcctcctctgccttgctggactggtatttgtgtctgaggctggccctacggtgagtgtttctgtgacatcccattcctacatttaagattcacgctaaatgaagtagaagtgactccttccagctttgccaaccagcttttattactagggcaagggtacccagcatctatttttaatataattaattcaaacttcaaaaagaatgaagttccactgagcttactgagctgggacttgaactctgagcattctacctcattgctttggtgcattaggtttgtaatatctggtacctctgtttcctcagatagatgatagaaataaagatatgatattaaggaagctgttaatactgaattttcagaaaagtatccctccataaaatgtatttgggggacaaactgcaggagattatattctggccctatagttattcaaaacgtatttattgattaatctttaaaaggcttagtgaacaatattctagtcagatatctaattcttaaatcctctagaagaattaactaatactataaaatgggtctggatgtagttctgacattattttataacaactggtaagagggagtgactatagcaacaactaaaatgatctcaggaaaacctgtttggccctatgtatggtacattacatcttttcagtaattccactcaaatggagacttttaacaaagcaactgttctcaggggacctattttctcccttaaaattcattatacacatccctggttgatagcagtgtgtctggaggcagaaaccattcttgctttggaaacaattacgtctgtgttatactgagtagggaagctcattaattgtcgacacttacgttcctgataatgggatcagtgtgtaattcttgtttcgctccagatttctaataccacaaagaataaatcctttcactctgatcaattttgttaacttctcacgtgtcttctctacacccagggcaccggtgaatccaagtgtcctctgatggtcaaagttctagatgctgtccgaggcagtcctgccatcaatgtggccgtgcatgtgttcagaaaggctgctgatgacacctgggagccatttgcctctgggtaagttgccaaagaaccctcccacaggacttggttttatcttcccgtttgcccctcacttggtagagagaggctcacatcatctgctaaagaatttacaagtagattgaaaaacgtaggcagaggtcaagtatgccctctgaaggatgccctctttttgttttgcttagctaggaagtgaccaggaacctgagcatcatttaggggcagacagtagagaaaagaaggaatcagaactcctctcctctagctgtggtttgcaacccttttgggtcacagaacactttatgtaggtgatgaaaagtaaacattctatgcccagaaaaaatgcacagatacacacacatacaaaatcatatatgtgattttaggagtttcacagattccctggtgtccctgggtaacaccaaagctaagtgtccttgtcttagaattttaggaaaaggtataatgtgtattaacccattaacaaaaggaaaggaattcagaaatattattaaccaggcatctgtctgtagttaatatggatcacccaaaacccaaggcttttgcctaatgaacactttggggcacctactgtgtgcaaggctgggggctgtcaagctcagttaaaaaaaaaaagatagaagagatggatccatgaggcaaagtacagccccaggctaatcccacgatcacccgacttcatgtccaagagtggcttctcaccttcattagccagttcacaattttcatggagtttttctacctgcactagcaaaaacttcaaggaaaatacatattaataaatctaagcaaagtgaccagaagacagagcaatcaggagaccctttgcatccagcagaagaggaactgctaagtatttacatctccacagagaagaatttctgttgggttttaattgaaccccaagaaccacatgattcttcaaccattattgggaagatcattttcttaggtctggttttaactggctttttatttgggaattcatttatgtttatataaaatgccaagcataacatgaaaagtggttacaggactattctaagggagagacagaatggacaccaaaaatattccaatgttcttgtgaatcttttccttgcaccaggacaaaaaaaaaaagaagtgaaaagaagaaaggaggaggggcataatcagagtcagtaaagacaactgctatttttatctatcgtagctgttgcagtcaaatgggaagcaatttccaacattcaactatggagctggtacttacatggaaatagaagttgcctagtgtttgttgctggcaaagagttatcagagaggttaaatatataaaagggaaaagagtcagatacaggttcttcttcctactttaggttttccactgtgtgtgcaaatgatactccctggtggtgtgcagatgcctcaaagctatcctcacaccacaagggagaggagcgagatcctgctgtcctggagaagtgcagagttagaacagctgtggccacttgcatccaatcatcaatcttgaatcacagggactctttcttaagtaaacattatacctggccgggcacggtggctcacgcctgtaatcccagcactttgggatgccaaagtgggcatatcatctgaggtcaggagttcaagaccagcctggccaacatggcaaaactccgtctttatgaaaaatacaaaaattagccaggcatggtggcaggcgcctgtaatcccagctaattgggaggctgaggctggagaatcccttgaatctaggaggcagaggttgcagtgagctgagatcgtgccattgcactccagcctgggtgacaagagtaaaactctgtctcaaaaaaaaaaaattatacctacattctcttcttatcagagaaaaaaatctacagtgagcttttcaaaaagtttttacaaactttttgccatttaatttcagttaggagttttccctacttctgacttagttgaggggaaatgttcataacatgtttataacatgtttatgtgtgttagttggtgggggtgtattactttgccatgccatttgtttcctccatgcgtaacttaatccagactttcacaccttataggaaaaccagtgagtctggagagctgcatgggctcacaactgaggaggaatttgtagaagggatatacaaagtggaaatagacaccaaatcttactggaaggcacttggcatctccccattccatgagcatgcagaggtgagtatacagaccttcgagggttgttttggttttggtttttgcttttggcattccaggaaatgcacagttttactcagtgtaccacagaaatgtcctaaggaaggtgatgaatgaccaaaggttccctttcctattatacaagaaaaaattcacaacactctgagaagcaaatttctttttgactttgatgaaaatccacttagtaacatgacttgaacttacatgaaactactcatagtctattcattccactttatatgaatattgatgtatctgctgttgaaataatagtttatgaggcagccctccagaccccacgtagagtgtatgtaacaagagatgcaccattttatttctcgaaaacccgtaacattcttcattccaaaacacatctggcttctcggaggtctggacaagtgattcttggcaacacatacctatagagacaataaaatcaaagtaataatggcaacacaatagataacatttaccaagcatacaccatgtggcagacacaattataagtgttttccatatttaacctacttaatcctcaggaataagccactgaggtcagtcctattattatccccatcttatagatgaagaaaatgaggcaccaggaagtcaaataacttgtcaaaggtcacaagactaggaaatacacaagtagaaatgtttacaattaaggcccaggctgggtttgccctcagttctgctatgcctcgcattatgccccaggaaactttttcccttgtgaaagccaagcttaaaaaaagaaaagccacatttgtaacgtgctctgttcccctgcctatggtgaggatcttcaaacagttatacatggacccagtccccctgccttctccttaatttcttaagtcatttgaaacagatggctgtcatggaaatagaatccagacatgttggtcagagttaaagatcaactaattccatcaaaaatagctcggcatgaaagggaactattctctggcttagtcatggatgagactttcaattgctataaagtggttcctttattagacaatgttaccagggaaacaacaggggtttgtttgacttctggggcccacaagtcaacaagagagccccatctaccaaggagcatgtccctgactacccctcagccagcagcaagacatggaccccagtcagggcaggagcagggtttcggcggcgcccagcacaagacattgcccctagagtctcagcccctaccctcgagtaatagatctgcctacctgagactgttgtttgcccaagagctgggtctcagcctgatgggaaccatataaaaaggttcactgacatactgcccacatgttgttctctttcattagatcttagcttccttgtctgctcttcattcttgcagtattcattcaacaaacattaaaaaaaaaaaaaagcattctatgtgtggaacactctgctagatgctgtggatttagaaatgaaaatacatcccgacccttggaatggaagggaaaggactgaagtaagacagattaagcaggaccgtcagcccagcttgaagcccagataaatacggagaacaagagagagcgagtagtgagagatgagtcccaatgcctcactttggtgacgggtgcgtggtgggcttcatgcagcttcttctgataaatgcctccttcagaactggtcaactctaccttggccagtgacccaggtggtcatagtagatttaccaagggaaaatggaaacttttattaggagctcttaggcctcttcacttcatggatttttttttcctttttttttgagatggagttttgccctgtcacccaggctggaatgcagtggtgcaatctcagctcactgcaacctccgcctcccaggttcaagcaattctcctgcctcagcctcccgagtagctgggactacaggtgtgcgccaccacaccaggctaatttttgtattttttgtaaagacaggttttcaccacgttggccaggctggtctgaactccagacctcaggtgattcacctgtctcagcctcccaaagtgctgggattacaggtgtgagccaccgtgcccggctacttcatggatttttgattacagattatgcctcttacaatttttaagaagaatcaagtgggctgaaggtcaatgtcaccataagacaaaagacatttttattagttgattctagggaattggccttaaggggagccctttcttcctaagagattcttaggtgattctcacttcctcttgccccagtattatttttgtttttggtatggctcactcagatccttttttcctcctatccctaagtaatccgggtttctttttcccatatttagaacaaaatgtatttatgcagagtgtgtccaaacctcaacccaaggcctgtatacaaaataaatcaaattaaacacatctttactgtcttctacctctttcctgacctcaatatatcccaacttgcctcactctgagaaccaaggctgtcccagcacctgagtcgcagatattctactgatttgacagaactgtgtgactatctggaacagcattttgatccacaatttgcccagttacaaagcttaaatgagctctagtgcatgcatatatatttcaaaattccaccatgatcttccacactctgtattgtaaatagagccctgtaatgcttttacttcgtatttcattgcttgttatacataaaaatatacttttcttcttcatgttagaaaatgcaaagaataggagggtgggggaatctctgggcttggagacaggagacttgccttcctactatggttccatcagaatgtagactgggacaatacaataattcaagtctggtttgctcatctgtaaattgggaagaatgtttccagctccagaatgctaaatctctaagtctgtggttggcagccactattgcagcagctcttcaatgactcaatgcagttttgcattctccctaccttttttttctaaaaccaataaaatagatacagcctttaggctttctgggatttcccttagtcaagctagggtcatcctgactttcggcgtgaatttgcaaaacaagacctgactctgtactcctgctctaaggactgtgcatggttccaaaggcttagcttgccagcatatttgagctttttccttctgttcaaactgttccaaaatataaaagaataaaattaattaagttggcactggacttccggtggtcagtcatgtgtgtcatctgtcacgtttttcgggctctggtggaaatggatctgtctgtcttctctcataggtggtattcacagccaacgactccggcccccgccgctacaccattgccgccctgctgagcccctactcctattccaccacggctgtcgtcaccaatcccaaggaatgagggacttctcctccagtggacctgaaggacgagggatgggatttcatgtaaccaagagtattccatttttactaaagcagtgttttcacctcatatgctatgttagaagtccaggcagagacaataaaacattcctgtgaaaggcacttttcattccactttaacttgattttttaaattcccttattgtcccttccaaaaaaaagagaatcaaaattttacaaagaatcaaaggaattctagaaagtatctgggcagaacgctaggagagatccaaatttccattgtcttgcaagcaaagcacgtattaaatatgatctgcagccattaaaaagacacattctgtaaatgagagagccttattttcctgtaaccttcagcaaatagcaaaagacacattccaagggcccacttctttactgtgggca

SEQ ID NO: 19 - DNA, 6208 bp, Homo sapiens
  source 1..6208: mol_type = other DNA
ggcaccggtgaatccaagtgtcctctgatggtcaaagttctagatgctgtccgaggcagtcctgccatcaatgtggccgtgcatgtgttcagaaaggctgctgatgacacctgggagccatttgcctctgggtaagttgccaaagaaccctcccacaggacttggttttatcttcccgtttgcccctcacttggtagagagaggctcacatcatctgctaaagaatttacaagtagattgaaaaacgtaggcagaggtcaagtatgccctctgaaggatgccctctttttgttttgcttagctaggaagtgaccaggaacctgagcatcatttaggggcagacagtagagaaaagaaggaatcagaactcctctcctctagctgtggtttgcaacccttttgggtcacagaacactttatgtaggtgatgaaaagtaaacattctatgcccagaaaaaatgcacagatacacacacatacaaaatcatatatgtgattttaggagtttcacagattccctggtgtccctgggtaacaccaaagctaagtgtccttgtcttagaattttaggaaaaggtataatgtgtattaacccattaacaaaaggaaaggaattcagaaatattattaaccaggcatctgtctgtagttaatatggatcacccaaaacccaaggcttttgcctaatgaacactttggggcacctactgtgtgcaaggctgggggctgtcaagctcagttaaaaaaaaaaagatagaagagatggatccatgaggcaaagtacagccccaggctaatcccacgatcacccgacttcatgtccaagagtggcttctcaccttcattagccagttcacaattttcatggagtttttctacctgcactagcaaaaacttcaaggaaaatacatattaataaatctaagcaaagtgaccagaagacagagcaatcaggagaccctttgcatccagcagaagaggaactgctaagtatttacatctccacagagaagaatttctgttgggttttaattgaaccccaagaaccacatgattcttcaaccattattgggaagatcattttcttaggtctggttttaactggctttttatttgggaattcatttatgtttatataaaatgccaagcataacatgaaaagtggttacaggactattctaagggagagacagaatggacaccaaaaatattccaatgttcttgtgaatcttttccttgcaccaggacaaaaaaaaaaagaagtgaaaagaagaaaggaggaggggcataatcagagtcagtaaagacaactgctatttttatctatcgtagctgttgcagtcaaatgggaagcaatttccaacattcaactatggagctggtacttacatggaaatagaagttgcctagtgtttgttgctggcaaagagttatcagagaggttaaatatataaaagggaaaagagtcagatacaggttcttcttcctactttaggttttccactgtgtgtgcaaatgatactccctggtggtgtgcagatgcctcaaagctatcctcacaccacaagggagaggagcgagatcctgctgtcctggagaagtgcagagttagaacagctgtggccacttgcatccaatcatcaatcttgaatcacagggactctttcttaagtaaacattatacctggccgggcacggtggctcacgcctgtaatcccagcactttgggatgccaaagtgggcatatcatctgaggtcaggagttcaagaccagcctggccaacatggcaaaactccgtctttatgaaaaatacaaaaattagccaggcatggtggcaggcgcctgtaatcccagctaattgggaggctgaggctggagaatcccttgaatctaggaggcagaggttgcagtgagctgagatcgtgccattgcactccagcctgggtgacaagagtaaaactctgtctcaaaaaaaaaaaattatacctacattctcttcttatcagagaaaaaaatctacagtgagcttttcaaaaagtttttacaaactttttgccatttaatttcagttaggagttttccctacttctgacttagttgaggggaaatgttcataacatgtttataacatgtttatgtgtgttagttggtgggggtgtattactttgccatgccatttgtttcctccatgcgtaacttaatccagactttcacaccttataggaaaaccagtgagtctggagagctgcatgggctcacaactgaggaggaatttgtagaagggatatacaaagtggaaatagacaccaaatcttactggaaggcacttggcatctccccattccatgagcatgcagaggtgagtatacagaccttcgagggttgttttggttttggtttttgcttttggcattccaggaaatgcacagttttactcagtgtaccacagaaatgtcctaaggaaggtgatgaatgaccaaaggttccctttcctattatacaagaaaaaattcacaacactctgagaagcaaatttctttttgactttgatgaaaatccacttagtaacatgacttgaacttacatgaaactactcatagtctattcattccactttatatgaatattgatgtatctgctgttgaaataatagtttatgaggcagccctccagaccccacgtagagtgtatgtaacaagagatgcaccattttatttctcgaaaacccgtaacattcttcattccaaaacacatctggcttctcggaggtctggacaagtgattcttggcaacacatacctatagagacaataaaatcaaagtaataatggcaacacaatagataacatttaccaagcatacaccatgtggcagacacaattataagtgttttccatatttaacctacttaatcctcaggaataagccactgaggtcagtcctattattatccccatcttatagatgaagaaaatgaggcaccaggaagtcaaataacttgtcaaaggtcacaagactaggaaatacacaagtagaaatgtttacaattaaggcccaggctgggtttgccctcagttctgctatgcctcgcattatgccccaggaaactttttcccttgtgaaagccaagcttaaaaaaagaaaagccacatttgtaacgtgctctgttcccctgcctatggtgaggatcttcaaacagttatacatggacccagtccccctgccttctccttaatttcttaagtcatttgaaacagatggctgtcatggaaatagaatccagacatgttggtcagagttaaagatcaactaattccatcaaaaatagctcggcatgaaagggaactattctctggcttagtcatggatgagactttcaattgctataaagtggttcctttattagacaatgttaccagggaaacaacaggggtttgtttgacttctggggcccacaagtcaacaagagagccccatctaccaaggagcatgtccctgactacccctcagccagcagcaagacatggaccccagtcagggcaggagcagggtttcggcggcgcccagcacaagacattgcccctagagtctcagcccctaccctcgagtaatagatctgcctacctgagactgttgtttgcccaagagctgggtctcagcctgatgggaaccatataaaaaggttcactgacatactgcccacatgttgttctctttcattagatcttagcttccttgtctgctcttcattcttgcagtattcattcaacaaacattaaaaaaaaaaaaaagcattctatgtgtggaacactctgctagatgctgtggatttagaaatgaaaatacatcccgacccttggaatggaagggaaaggactgaagtaagacagattaagcaggaccgtcagcccagcttgaagcccagataaatacggagaacaagagagagcgagtagtgagagatgagtcccaatgcctcactttggtgacgggtgcgtggtgggcttcatgcagcttcttctgataaatgcctccttcagaactggtcaactctaccttggccagtgacccaggtggtcatagtagatttaccaagggaaaatggaaacttttattaggagctcttaggcctcttcacttcatggatttttttttcctttttttttgagatggagttttgccctgtcacccaggctggaatgcagtggtgcaatctcagctcactgcaacctccgcctcccaggttcaagcaattctcctgcctcagcctcccgagtagctgggactacaggtgtgcgccaccacaccaggctaatttttgtattttttgtaaagacaggttttcaccacgttggccaggctggtctgaactccagacctcaggtgattcacctgtctcagcctcccaaagtgctgggattacaggtgtgagccaccgtgcccggctacttcatggatttttgattacagattatgcctcttacaatttttaagaagaatcaagtgggctgaaggtcaatgtcaccataagacaaaagacatttttattagttgattctagggaattggccttaaggggagccctttcttcctaagagattcttaggtgattctcacttcctcttgccccagtattatttttgtttttggtatggctcactcagatccttttttcctcctatccctaagtaatccgggtttctttttcccatatttagaacaaaatgtatttatgcagagtgtgtccaaacctcaacccaaggcctgtatacaaaataaatcaaattaaacacatctttactgtcttctacctctttcctgacctcaatatatcccaacttgcctcactctgagaaccaaggctgtcccagcacctgagtcgcagatattctactgatttgacagaactgtgtgactatctggaacagcattttgatccacaatttgcccagttacaaagcttaaatgagctctagtgcatgcatatatatttcaaaattccaccatgatcttccacactctgtattgtaaatagagccctgtaatgcttttacttcgtatttcattgcttgttatacataaaaatatacttttcttcttcatgttagaaaatgcaaagaataggagggtgggggaatctctgggcttggagacaggagacttgccttcctactatggttccatcagaatgtagactgggacaatacaataattcaagtctggtttgctcatctgtaaattgggaagaatgtttccagctccagaatgctaaatctctaagtctgtggttggcagccactattgcagcagctcttcaatgactcaatgcagttttgcattctccctaccttttttttctaaaaccaataaaatagatacagcctttaggctttctgggatttcccttagtcaagctagggtcatcctgactttcggcgtgaatttgcaaaacaagacctgactctgtactcctgctctaaggactgtgcatggttccaaaggcttagcttgccagcatatttgagctttttccttctgttcaaactgttccaaaatataaaagaataaaattaattaagttggcactggacttccggtggtcagtcatgtgtgtcatctgtcacgtttttcgggctctggtggaaatggatctgtctgtcttctctcataggtggtattcacagccaacgactccggcccccgccgctacaccattgccgccctgctgagcccctactcctattccaccacggctgtcgtcaccaatcccaaggaatgagggacttctcctccagtggacctgaaggacgagggatgggatttcatgtaaccaagagtattccatttttactaaagcagtgttttcacctcatatgctatgttagaagtccaggcagagacaataaaacattcctgtgaaaggcacttttcattccactttaacttgattttttaaattcccttattgtcccttccaaaaaaaagagaatcaaaattttacaaagaatcaaaggaattctagaaagtatctgggcagaacgctaggagagatccaaatttccattgtcttgcaagcaaagcacgtattaaatatgatctgcagccattaaaaagacacattctgtaaatgagagagccttattttcctgtaaccttcagcaaatagcaaaagacacattccaagggcccacttctttactgtgggca

SEQ ID NO: 20 - DNA, 8300 bp, Mus musculus
  source 1..8300: mol_type = other DNA
atggcttcccttcgactcttcctcctttgcctcgctggactggtatttgtgtctgaagctggccccgcggtgagtgatcctgtgagcgatccagacatggcagttagaccttagataaagaagaagtgccttcttccagatgtgagaactagagtactcagactctatatttaccattagactccaaagagaagagctggagtgcctctggctcttccttctattgctttagcgcattgggtctgtagtgctcagtctctggtgtccttagataataaagatatgagattaacatagaaataaagatataaaagggctggatgtatagtttagtggtccagtgtatgcctagtatgtgaaaagccttctgttcaacctctagcaatagaaaaacaagatatattctcggtggggctgttaatattgaattctcataaaatctttaatatatttagtatgcctattatgttgttatattttagttctttagctaatcaaaatgcattattgatctttctttgtctttttttggccaacactctattccagtctttgaaaaagtcctttaaaagagttaatcagtataattaaatgagtcaggaagtatgtgagggttattttacaaccagagggaattactatagcaacagctgattagaatgatctcaagaaaaagcccattctgtctttttgcaccatgcacctttcagtggctccattcagatggagaggcaaacagagcaatggctctcagagggcctattttccctttgaacattcattatccatatccctggtgcacagcagtgcatctgggggcagaaactgttcttgctttggaaacaatgctgtctatgtcatactggataaagaagctcattaattgtcaacacttatgttatcataatgggatcagcatgtacttttggttttgttccagagtctatcaccggaaagaacaagccggtttactctgacccatttcactgacatttctcttgtctcctctgtgcccagggtgctggagaatccaaatgtcctctgatggtcaaagtcctggatgctgtccgaggcagccctgctgtagacgtggctgtaaaagtgttcaaaaagacctctgagggatcctgggagccctttgcctctgggtaagcttgtagaaagcccaccatgggaccggttccaggttcccatttgctcttattcgtgttagattcagacacacacaacttaccagctagagggctcagagagagggctcaggggcgaagggcacgtattgctcttgtaagagacacaggtttaattcctagcaccagaatggcagctcataaccatctgaaactcacagtcttaggagatctgggtatctgacattctcttctacccaccatgtgtgtggtgcacaaattcacatgcaggcatcaaatcttataaacaacaacaaaaaaccaacaaacctggtagcaaaagaagattagaaggttaaacatatgagccgagagcttttgttttgttttgttttgttttgttttgtttacatttcaaatgttatcccctttctcggtccccctccccaaaccctctaccccattctctcctccccttcttctatgagggtgttccccaccaacccactcccaccttcctgctctcgaattcccctatactgggacatcaagccttcacagaatcaagggcctctcctcccattgatgcccgacaatgtcatcctctgctacctatgtggctggagccatgggtcccttcatgtatcctccttggttggtggtttagtctctgggaggtctgggggatctggttgattgatattattgttcttcctatgagattgcaaaccccttcagctccttcggtcctttaactcctccactggggaccccgagctcagtccaatggttggctgtgagcatccaccagcagaggcctttttttttttttttaacaaagctgctttattatgttgcttagagcatgaccaggaaccagagcacagtccaagactgaagggaggaaaagggggggagtcaataaccccactgtttcatagtggtttgcaacccttttatatcacagcccactttaggcaaataatgaaaattatagtctccagggacagagaagatggtgcaggaagtgaagtgcctgctcagaaaatgggggcttgaatgtgagttcccagactctgtgtaagatgcccagcatcgaagtgcatgcttataacaccagcctggaggtagaagcttagaaacaggggtaccctgaagttgcttgttcaccagtgtccctgaatgggtaggtgcatgtttggtgagagaccctgtctcaaaaatcaaggtgtaggataattgaaaatacctagctttgagcttagatcatgcaaatgtgtacacacactcacacacaccacacacacaaaaaaatgcagagacagagagatacagagagacagagagatacagagacagagacagagagaaaaggagaaagtaaaaaacaaataatttaaagacccatggccacaaagaggctcaaagacaagcacgtataaaaccatacacatgtaattttaggagttttcagattccctggtacccgtgggtgatgcacaagctttgaatcccagtcttaaaatcttacgaagaacgtgttcgtgtgtgctaatttattgatgagaggaaaggaattgacaaagtgcccttccggagcttcctgcattacccagactcagggtttttttaaatgtacactcagaacagagtagctctgtgcaagggtagcaaccacgaagcttaataagaaacatatcgtgagagatctgcaaggcaaatctaggggctgaccaatctcacagtcacccactagcatgtcaacacaacttcccacctgtgctagccacttagcaattttgtgttgttctgttttgtttttgtttttaacaaagcaatttcaaagagatttctaattcatctaaacaaacaaaccaaaaggaaaacagcaaagacgccctgagcacttagcagagcagctatgcagttatgactcctgggtggagactttatatcaggcttcaactgaatacctagaacctactagtgctcttcatcaatccttgggaaggtcattttcttttggtgctgttttgagtttctatttgttaatgtcttcataattatacacgtgttgagcacagcatgcaaagtgattaggggaatctagttggagtggaatggatacccaaatattcagactttcttgtgactcttctttcttgtacccacatcaaaaaaaaaaaaaatggagatgagacatggtcagagtcactaaaaccagctgctacttttaattacgtggggagcagtttctaacattgccattattgaactgatgctgcctgggtggaaatggaaatcacttagtatttcttgttggcaaagaattactgaatggattaaatttccaaagggagaagtcagttacaagtcttttctttgtttattaggctttctgctatgataaattacactacttccagaagttacccttaggccatgggacactggactatcactctgctgtcacaagagattacagagttagtcaaggcagcttgtgacaccttcagggactgtcataaacttccagcaagtcattaatcctgaatgcaatactgtgtgtgtgtgtctatgtgtgtttgtatgtctgtgtgtgtcttatgtctgtgtctctgtgtgtgtgtgtgtttgtgtgtgtgtgtgtatgtatgcctgtgtgtgtcttatgtctgtgtttgtgtgtctgtgtgtgtcttatgtctgtgtttgtatgtctgtgtgtgtctgtgtgtgtcttatgtctgtgtctctgtgtgtgtgtgtgtgtatgtatgtatgtatgtatgtatgtgtatgtgtttgcatctctctgtgtgtctgcgcttatatatttgtgtatgtgtttatgtgttcgcctttgtgcgttgttggggattgaatccaggggaatacaaatgttaagaaagaacgttaccactaagcttcacctgtaggccttaaagcttttctttcttttaaaaattgtaattaattcattttcagtcaggatctccacacctcgtccctgctgctctagaactcactatttaaacacaatcgccctcaaacctgcagcaaccctcccgcctctaccctgcgagcactagaataataacaggtgaccccacacgcctagattaagacctttaaggtaaacattttactatattttagtctcataagacaagatgctacaataaagctgtacataaagttccctcgaatttcttgctattttaactcaaacataaggatttcctcctttttgattcaggtaacagaaaaaatacacaggtacatacatgtacacacatgaacacacacgcatcacaaccacatatgcgcacgcttgtgtgatctatcatttaccatgccactgaactcttctttccccataaattcctctggacttgtgtgccctccaggaagaccgcggagtctggagagctgcacgggctcaccacagatgagaagtttgtagaaggagtgtacagagtagaactggacaccaaatcgtactggaagacacttggcatttccccgttccatgaattcgcggatgtaagtggacacaccaagttgtttggattttgtttttagtctcaggaaattcccttcgctcttgctgtacgatgggcatgagtggaaagtagattccacagccagaatccacagtgctgggaaagcaagccttctgaatttttctaaaactcatttagcaacatggcctgaacctgttcacactgcttatggtcagctaactatatttatgtaaatattcatttctctgttgaggaaatgttagtatttgcttttgaggcaacctccagataccatggagggcatgtcatagtcaaagagagggctccctatggtatttctctaaattctggcatttcctttattccaaagcacatctagtgtccccagaagtttgggtagacaattcttggcaacacagagaattacaacatgttcaaaacccaacagcttaatatctaaatcatcaagcaaacatcacatggcaaagggatttctgaatcaaaactgtttcatccttatgatcaacctatggaggtctagcctcgacttacacccattttaccaataagctaagagaagctaagttcctcatcaaggacacaaggctagcatgtgtgagcaagtgacagagttgccctctatgttggttagtgtgccttagccagtgtctcagtaagaaatggagctaaatcaaaacccaaggccaacagccaaaggcacatgagtaacctttgcttggcactgggctcagtttccctggctcctctcagtcctcagttcacagaggcagctgtcatgcaaatagaatccaagcttgttggtcagacctggagataacaaattccatcaaaaatagctcctcatgtgacctagtttgctgtctgttgctatgatacacaccatgaccgaaaagcaaccctggggagagaagggtttatttcatcttacagcttacagttcaccatggaggaaagccaggtgggaacctggaagtggaaattgaagcagagaccagaaaggaatgctgtttactggctggcttagctccttttcttatacagcttaggtctatgtgcccaggggatggtactgccgagcataggctgagcccgcctacatcaaccattagtcaaaaaaaggtccatagacttgcctacaggccaatctcatggaggcaataccccagtggagggtccctcttcgcaggttactctagtttgtgtcaagttgacaaaacctaaccacaaagcacaaacagggtctgcccttgtggcttagccatggatgacactctcagatgatggtgttaccagacaaaccagaggggctcaccaagagtctgccacctaccaaggtagtactctactcctcactgggcaccaacacccatattagctgggccagtacaggacccttgctgtttcctgcatgaattgtccatagaccctgggtctcagcctgccgggagtacctgtaagtagtcgcctcaaacacattattcctgttggaagacttgtctgattctcttttagaactcaatcaacaaacgtttttattttgttttggctttttggagacaagatctctcataggccagcctgacttgaatgtagctgaggatgacctgtgctgctaatcttctcgcctcttcctcccaagtggtaggataataggcataagacaccacagcagttttactccataccagggctctgaacccagactttaaacactctatcaactgattcacattcccaccccatcattcaacaaacatttgaaaaataaaacccttctgccttgagcactctgctaaatacagcctttgagtgcggagtatttcctcacaaccagggtccaagatgaccccatcatacataccacggaaaattaggagatgtttttaggtctctttgcttggggtaatttttatgtgtgtgtgtacacagccctgtgcgtgtgtgtgtgtgtgtgtgtgtgtgtgtacaggcacacacgtgtatgcatgtagaggctacataaaaaccttaggtgtcattctcaggcactctgttcaccccttcacacagcccgaacacacaaaatttgaggcattagcctggagctcaccagttaggctagactgacttgccagcagaccccaggctgtctccatctccccagctctgggattacaaactctatcataccagacatttttatacatattctgagcataaaattcatgtcttcaggctaacaagtcaagagcttaaatgactgagctctcttacgtggtggattttttttaaaactacataatatcttttttttttttttcacttctggggaagaaacaaatgagcctgagtgacaatgcgacagaaaagaaattttgaggagtgtgtgtgtctgtgtgtgtggtggcacatgcctctcatctaatgctagaggctacagtagaatgctcctgaattagtggccagccaaggccaagggctagggttgtaactcagtggcagagggcttgcctagcattcgcaggatttgatccatagcgctataaataataataaataaatacaacagtctaagatgattctccctttcatttatctggatgttatttttgtgttagttttactctgtcatccaatcattgtttgccctatatttggacatttaaaaaaaatctttattccaagtgtgttcaaagctgtatccaaaacctgtccaccaaatgagtccaatgacatacatcttctatattaccatctgttccagatttggctgactcccggcacctgggctgttgctgcacccatgtctcagatagtctagtgatttgagaagtgactagtaattgcaaaatccagactttgtccagaaacttctatgagctccaaaactttcatttacatttctgccagccacaaaccgcttgtgttgtggagagaaccctgtgatgtcttcccacagcatctcagccttgtttcttcccttaaaatattcatcttttcacattagaacatgcaaagggacagtgggagcgaaacccctggactgggacgcacgaagccttcctttctggtcaggctctcactgtagaaacttaggccggtttcagcatgcagtctgctggagaatggctcctgccaacattccaggtctggaagtttgtagtggagttgttgataaccactgttcgccacaggtcttttgtttgtgggtgtcagtgtttctactctcctgacttttatctgaacccaagaaagggaacaatagccttcaagctctctgtgactctgatctgaccagggccacccacactgcagaaggaaacttgcaaagagagacctgcaattctctaagagctccacacagctccaaagacttaggcagcatattttaatctaattattcgtcccccaaccccaccccagaggacagttagacaataaaaggaagattaccagcttagcatcctgtgaacactttgtctgcagctcctacctctgggctctgttagaactagctgtctctcctctctcctaggtggttttcacagccaacgactctggccatcgccactacaccatcgcagccctgctcagcccatactcctacagcaccacggctgtcgtcagcaacccccagaattga

SEQ ID NO: 21 - DNA, 24 bp, synthetic construct
  misc_feature 1..24: note = Synthetic
  source 1..24: mol_type = other DNA
cacagacaatcagacgtaccagta

SEQ ID NO: 22 - DNA, 20 bp, synthetic construct
  misc_feature 1..20: note = Synthetic
  source 1..20: mol_type = other DNA
ccagctttgccagtttacga

SEQ ID NO: 23 - DNA, 18 bp, synthetic construct
  misc_feature 1..18: note = Synthetic
  source 1..18: mol_type = other DNA
ttggacggttgccctctt

SEQ ID NO: 24 - DNA, 22 bp, synthetic construct
  misc_feature 1..22: note = Synthetic
  source 1..22: mol_type = other DNA
gatggcttcccttcgactcttc

SEQ ID NO: 25 - DNA, 25 bp, synthetic construct
  misc_feature 1..25: note = Synthetic
  source 1..25: mol_type = other DNA
cactgacatttctcttgtctcctct

SEQ ID NO: 26 - DNA, 21 bp, synthetic construct
  misc_feature 1..21: note = Synthetic
  source 1..21: mol_type = other DNA
gggctcaccacagatgagaag

SEQ ID NO: 27 - DNA, 20 bp, synthetic construct
  misc_feature 1..20: note = Synthetic
  source 1..20: mol_type = other DNA
cactgttcgccacaggtctt

SEQ ID NO: 28 - DNA, 20 bp, synthetic construct
  misc_feature 1..20: note = Synthetic
  source 1..20: mol_type = other DNA
gctcagcccatactcctaca

SEQ ID NO: 29 - DNA, 18 bp, synthetic construct
  misc_feature 1..18: note = Synthetic
  source 1..18: mol_type = other DNA
gcccaggaggaccaggat

SEQ ID NO: 30 - DNA, 20 bp, synthetic construct
  misc_feature 1..20: note = Synthetic
  source 1..20: mol_type = other DNA
ggcaacttgcttgaggaaga

SEQ ID NO: 31 - DNA, 20 bp, synthetic construct
  misc_feature 1..20: note = Synthetic
  source 1..20: mol_type = other DNA
gcagcaacccagcttcactt

SEQ ID NO: 32 - DNA, 19 bp, synthetic construct
  misc_feature 1..19: note = Synthetic
  source 1..19: mol_type = other DNA
actgagctgggacttgaac

SEQ ID NO: 33 - DNA, 19 bp, synthetic construct
  misc_feature 1..19: note = Synthetic
  source 1..19: mol_type = other DNA
tgcctcactctgagaacca

SEQ ID NO: 34 - DNA, 19 bp, synthetic construct
  misc_feature 1..19: note = Synthetic
  source 1..19: mol_type = other DNA
ggtggagaggctattcggc

SEQ ID NO: 35 - DNA, 18 bp, synthetic construct
  misc_feature 1..18: note = Synthetic
  source 1..18: mol_type = other DNA
ggccgtgcatgtgttcag

SEQ ID NO: 36 - DNA, 23 bp, synthetic construct
  misc_feature 1..23: note = Synthetic
  source 1..23: mol_type = other DNA
ggttcccatttgctcttattcgt

SEQ ID NO: 37 - DNA, 23 bp, synthetic construct
  misc_feature 1..23: note = Synthetic
  source 1..23: mol_type = other DNA
cccacactgcagaaggaaacttg

SEQ ID NO: 38 - DNA, 23 bp, synthetic construct
  misc_feature 1..23: note = Synthetic
  source 1..23: mol_type = other DNA
ggttcccatttgctcttattcgt

SEQ ID NO: 39 - DNA, 22 bp, synthetic construct
  misc_feature 1..22: note = Synthetic
  source 1..22: mol_type = other DNA
ccagcttagcatcctgtgaaca

SEQ ID NO: 40 - DNA, 20 bp, synthetic construct
  misc_feature 1..20: note = Synthetic
  source 1..20: mol_type = other DNA
ggcaacttgcttgaggaaga

SEQ ID NO: 41 - DNA, 22 bp, synthetic construct
  misc_feature 1..22: note = Synthetic
  source 1..22: mol_type = other DNA
tgtggagttcagtagtgtggag

SEQ ID NO: 42 - DNA, 25 bp, synthetic construct
  misc_feature 1..25: note = Synthetic
  source 1..25: mol_type = other DNA
cactgacatttctcttgtctcctct

SEQ ID NO: 43 - DNA, 23 bp, synthetic construct
  misc_feature 1..23: note = Synthetic
  source 1..23: mol_type = other DNA
gggacatctcggtttcctgactt

SEQ ID NO: 44 - DNA, 22 bp, synthetic construct
  misc_feature 1..22: note = Synthetic
  source 1..22: mol_type = other DNA
tccacactactgaactccacaa

SEQ ID NO: 45 - DNA, 21 bp, synthetic construct
  misc_feature 1..21: note = Synthetic
  source 1..21: mol_type = other DNA
cggaacactcgctctacgaaa

SEQ ID NO: 46 - DNA, 18 bp, synthetic construct
  misc_feature 1..18: note = Synthetic
  source 1..18: mol_type = other DNA
gggccagcttcagacaca

SEQ ID NO: 47 - DNA, 22 bp, synthetic construct
  misc_feature 1..22: note = Synthetic
  source 1..22: mol_type = other DNA
cccagggtgctggagaatccaa

SEQ ID NO: 48 - DNA, 22 bp, synthetic construct
  misc_feature 1..22: note = Synthetic
  source 1..22: mol_type = other DNA
gccaagtgtcttccagtacgat

SEQ ID NO: 49 - DNA, 21 bp, synthetic construct
  misc_feature 1..21: note = Synthetic
  source 1..21: mol_type = other DNA
gttccctttcttgggttcaga

SEQ ID NO: 50 - DNA, 23 bp, synthetic construct
  misc_feature 1..23: note = Synthetic
  source 1..23: mol_type = other DNA
gatgctactgctttggcaagatc

SEQ ID NO: 51 - DNA, 20 bp, synthetic construct
  misc_feature 1..20: note = Synthetic
  source 1..20: mol_type = other DNA
cctgagctgctaacacggtt

SEQ ID NO: 52 - DNA, 23 bp, synthetic construct
  misc_feature 1..23: note = Synthetic
  source 1..23: mol_type = other DNA
agctacagaccatgcttagtgta

SEQ ID NO: 53 - DNA, 24 bp, synthetic construct
  misc_feature 1..24: note = Synthetic
  source 1..24: mol_type = other DNA
tgccagtttaggaggaatatgttc

SEQ ID NO: 54 - DNA, 25 bp, synthetic construct
  misc_feature 1..25: note = Synthetic
  source 1..25: mol_type = other DNA
ctgaggaaacagaggtaccagatat

SEQ ID NO: 55 - DNA, 24 bp, synthetic construct
  misc_feature 1..24: note = Synthetic
  source 1..24: mol_type = other DNA
agtcacacagttctgtcaaatcag

SEQ ID NO: 56 - DNA, 17 bp, synthetic construct
  misc_feature 1..17: note = Synthetic
  source 1..17: mol_type = other DNA
gaacacggcggcatcag

SEQ ID NO: 57 - DNA, 20 bp, synthetic construct
  misc_feature 1..20: note = Synthetic
  source 1..20: mol_type = other DNA
tcctgtgggagggttctttg

SEQ ID NO: 58 - DNA, 20 bp, synthetic construct
  misc_feature 1..20: note = Synthetic
  source 1..20: mol_type = other DNA
ccctctctctgagccctcta

SEQ ID NO: 59 - DNA, 21 bp, synthetic construct
  misc_feature 1..21: note = Synthetic
  source 1..21: mol_type = other DNA
gctgcctaagtctttggagct

SEQ ID NO: 60 - DNA, 20 bp, synthetic construct
  misc_feature 1..20: note = Synthetic
  source 1..20: mol_type = other DNA
ccctctctctgagccctcta

SEQ ID NO: 61 - DNA, 25 bp, synthetic construct
  misc_feature 1..25: note = Synthetic
  source 1..25: mol_type = other DNA
gagaggagagacagctagttctaac

SEQ ID NO: 62 - DNA, 23 bp, synthetic construct
  misc_feature 1..23: note = Synthetic
  source 1..23: mol_type = other DNA
agctacagaccatgcttagtgta

SEQ ID NO: 63 - DNA, 22 bp, synthetic construct
  misc_feature 1..22: note = Synthetic
  source 1..22: mol_type = other DNA
gccctcttcatacaggaatcac

SEQ ID NO: 64 - DNA, 19 bp, synthetic construct
  misc_feature 1..19: note = Synthetic
  source 1..19: mol_type = other DNA
cggacagcatccaggactt

SEQ ID NO: 65 - DNA, 26 bp, synthetic construct
  misc_feature 1..26: note = Synthetic
  source 1..26: mol_type = other DNA
tcatgtaatctggcttcagagtggga

SEQ ID NO: 66 - DNA, 27 bp, synthetic construct
  misc_feature 1..27: note = Synthetic
  source 1..27: mol_type = other DNA
tgggaggcaattcttagtttcaatgga

SEQ ID NO: 67 - DNA, 23 bp, synthetic construct
  misc_feature 1..23: note = Synthetic
  source 1..23: mol_type = other DNA
tcccaaaggtgtctgtctgcaca

SEQ ID NO: 68 - DNA, 22 bp, synthetic construct
  misc_feature 1..22: note = Synthetic
  source 1..22: mol_type = other DNA
ctcctttgcctcgctggactgg

SEQ ID NO: 69 - DNA, 19 bp, synthetic construct
  misc_feature 1..19: note = Synthetic
  source 1..19: mol_type = other DNA
cggacagcatccaggactt

SEQ ID NO: 70 - DNA, 29 bp, synthetic construct
  misc_feature 1..29: note = Synthetic
  source 1..29: mol_type = other DNA
agaaggagtgtacagagtagaactggaca

SEQ ID NO: 71 - DNA, 27 bp, synthetic construct
  misc_feature 1..27: note = Synthetic
  source 1..27: mol_type = other DNA
tgtttgtgggtgtcagtgtttctactc

SEQ ID NO: 72 - DNA, 21 bp, synthetic construct
  misc_feature 1..21: note = Synthetic
  source 1..21: mol_type = other DNA
caccacggctgtcgtcagcaa

SEQ ID NO: 73 - DNA, 23 bp, synthetic construct
  misc_feature 1..23: note = Synthetic
  source 1..23: mol_type = other DNA
cttgccaaagcagtagcatccca

SEQ ID NO: 74 - DNA, 23 bp, synthetic construct
  misc_feature 1..23: note = Synthetic
  source 1..23: mol_type = other DNA
aggtcagaaagcagagtggacca

SEQ ID NO: 75 - DNA, 23 bp, synthetic construct
  misc_feature 1..23: note = Synthetic
  source 1..23: mol_type = other DNA
cccaggcaattcctaccttccca

SEQ ID NO: 76 - DNA, 28 bp, synthetic construct
  misc_feature 1..28: note = Synthetic
  source 1..28: mol_type = other DNA
tctgagcattctacctcattgctttggt

SEQ ID NO: 77 - DNA, 23 bp, synthetic construct
  misc_feature 1..23: note = Synthetic
  source 1..23: mol_type = other DNA
aggctgtcccagcacctgagtcg

SEQ ID NO: 78 - DNA, 23 bp, synthetic construct
  misc_feature 1..23: note = Synthetic
  source 1..23: mol_type = other DNA
tgggcacaacagacaatcggctg

SEQ ID NO: 79 - DNA, 23 bp, synthetic construct
  misc_feature 1..23: note = Synthetic
  source 1..23: mol_type = other DNA
aaggctgctgatgacacctggga

SEQ ID NO: 80 - DNA, 27 bp, synthetic construct
  misc_feature 1..27: note = Synthetic
  source 1..27: mol_type = other DNA
agattcagacacacacaacttaccagc

SEQ ID NO: 81 - DNA, 28 bp, synthetic construct
  misc_feature 1..28: note = Synthetic
  source 1..28: mol_type = other DNA
agacctgcaattctctaagagctccaca

SEQ ID NO: 82 - DNA, 27 bp, synthetic construct
  misc_feature 1..27: note = Synthetic
  source 1..27: mol_type = other DNA
agattcagacacacacaacttaccagc

SEQ ID NO: 83 - DNA, 24 bp, synthetic construct
  misc_feature 1..24: note = Synthetic
  source 1..24: mol_type = other DNA
ttgtctgcagctcctacctctggg

SEQ ID NO: 84 - DNA, 23 bp, synthetic construct
  misc_feature 1..23: note = Synthetic
  source 1..23: mol_type = other DNA
aggtcagaaagcagagtggacca

SEQ ID NO: 85 - DNA, 29 bp, synthetic construct
  misc_feature 1..29: note = Synthetic
  source 1..29: mol_type = other DNA
ttgacatgtgtgggtgagagattttactg

SEQ ID NO: 86 - DNA, 22 bp, synthetic construct
  misc_feature 1..22: note = Synthetic
  source 1..22: mol_type = other DNA
cccagggtgctggagaatccaa

SEQ ID NO: 87 - RNA, 16 nt, synthetic construct
  misc_feature 1..16: note = Synthetic
  source 1..16: mol_type = other RNA
gttttagagctatgct

SEQ ID NO: 88 - RNA, 67 nt, synthetic construct
  misc_feature 1..67: note = Synthetic
  source 1..67: mol_type = other RNA
agcatagcaagttaaaataaggctagtccgttatcaacttgaaaaagtggcaccgagtcggtgcttt

SEQ ID NO: 89 - RNA, 77 nt, synthetic construct
  misc_feature 1..77: note = Synthetic
  source 1..77: mol_type = other RNA
gttttagagctagaaatagcaagttaaaataaggctagtccgttatcaacttgaaaaagtggcaccgagtcggtgct

SEQ ID NO: 90 - DNA, 444 bp, synthetic construct
  misc_feature 1..444: note = Synthetic
  source 1..444: mol_type = other DNA
atggcttctcatcgtctgctcctcctctgccttgctggactggtatttgtgtctgaggctggccctacgggcaccggtgaatccaagtgtcctctgatggtcaaagttctagatgctgtccgaggcagtcctgccatcaatgtggccgtgcatgtgttcagaaaggctgctgatgacacctgggagccatttgcctctgggaaaaccagtgagtctggagagctgcatgggctcacaactgaggaggaatttgtagaagggatatacaaagtggaaatagacaccaaatcttactggaaggcacttggcatctccccattccatgagcatgcagaggtggtattcacagccaacgactccggcccccgccgctacaccattgccgccctgctgagcccctactcctattccaccacggctgtcgtcaccaatcccaaggaatga

SEQ ID NO: 91 - DNA, 444 bp, synthetic construct
  misc_feature 1..444: note = Synthetic
  source 1..444: mol_type = other DNA
atggcttcccttcgactcttcctcctttgcctcgctggactggtatttgtgtctgaagctggccccgcgggcaccggtgaatccaagtgtcctctgatggtcaaagttctagatgctgtccgaggcagtcctgccatcaatgtggccgtgcatgtgttcagaaaggctgctgatgacacctgggagccatttgcctctgggaaaaccagtgagtctggagagctgcatgggctcacaactgaggaggaatttgtagaagggatatacaaagtggaaatagacaccaaatcttactggaaggcacttggcatctccccattccatgagcatgcagaggtggtattcacagccaacgactccggcccccgccgctacaccattgccgccctgctgagcccctactcctattccaccacggctgtcgtcaccaatcccaaggaatga

SEQ ID NO: 92 - DNA, 444 bp, synthetic construct
  misc_feature 1..444: note = Synthetic
  source 1..444: mol_type = other DNA
atggcttcccttcgactcttcctcctttgcctcgctggactggtatttgtgtctgaagctggccccgcgggtgctggagaatccaaatgtcctctgatggtcaaagtcctggatgctgtccgaggcagccctgctgtagacgtggctgtaaaagtgttcaaaaagacctctgagggatcctgggagccctttgcctctgggaagaccgcggagtctggagagctgcacgggctcaccacagatgagaagtttgtagaaggagtgtacagagtagaactggacaccaaatcgtactggaagacacttggcatttccccgttccatgaattcgcggatgtggttttcacagccaacgactctggccatcgccactacaccatcgcagccctgctcagcccatactcctacagcaccacggctgtcgtcagcaacccccagaattga

SEQ ID NO: 93 - DNA, 4176 bp, synthetic construct
  misc_feature 1..4176: note = Synthetic
  misc_feature 1..3: note = Start Codon
  misc_feature 10..30: note = 5' NLS
  misc_feature 4126..4173: note = 3' NLS
  misc_feature 4174..4176: note = Stop Codon
  source 1..4176: mol_type = other DNA
atggacaagcccaagaaaaagcggaaagtgaagtacagcatcggcctggacatcggcaccaactctgtgggctgggccgtgatcaccgacgagtacaaggtgcccagcaagaaattcaaggtgctgggcaacaccgacaggcacagcatcaagaagaacctgatcggcgccctgctgttcgacagcggcgaaacagccgaggccaccagactgaagagaaccgccagaagaagatacaccaggcggaagaacaggatctgctatctgcaagagatcttcagcaacgagatggccaaggtggacgacagcttcttccacagactggaagagtccttcctggtggaagaggacaagaagcacgagagacaccccatcttcggcaacatcgtggacgaggtggcctaccacgagaagtaccccaccatctaccacctgagaaagaaactggtggacagcaccgacaaggccgacctgagactgatctacctggccctggcccacatgatcaagttcagaggccacttcctgatcgagggcgacctgaaccccgacaacagcgacgtggacaagctgttcatccagctggtgcagacctacaaccagctgttcgaggaaaaccccatcaacgccagcggcgtggacgccaaggctatcctgtctgccagactgagcaagagcagaaggctggaaaatctgatcgcccagctgcccggcgagaagaagaacggcctgttcggcaacctgattgccctgagcctgggcctgacccccaacttcaagagcaacttcgacctggccgaggatgccaaactgcagctgagcaaggacacctacgacgacgacctggacaacctgctggcccagatcggcgaccagtacgccgacctgttcctggccgccaagaacctgtctgacgccatcctgctgagcgacatcctgagagtgaacaccgagatcaccaaggcccccctgagcgcctctatgatcaagagatacgacgagcaccaccaggacctgaccctgctgaaagctctcgtgcggcagcagctgcctgagaagtacaaagaaatcttcttcgaccagagcaagaacggctacgccggctacatcgatggcggcgctagccaggaagagttctacaagttcatcaagcccatcctggaaaagatggacggcaccgaggaactgctcgtgaagctgaacagagaggacctgctgagaaagcagagaaccttcgacaacggcagcatcccccaccagatccacctgggagagctgcacgctatcctgagaaggcaggaagatttttacccattcctgaaggacaaccgggaaaagatcgagaagatcctgaccttcaggatcccctactacgtgggccccctggccagaggcaacagcagattcgcctggatgaccagaaagagcgaggaaaccatcaccccctggaacttcgaggaagtggtggacaagggcgccagcgcccagagcttcatcgagagaatgacaaacttcgataagaacctgcccaacgagaaggtgctgcccaagcacagcctgctgtacgagtacttcaccgtgtacaacgagctgaccaaagtgaaatacgtgaccgagggaatgagaaagcccgccttcctgagcggcgagcagaaaaaggccatcgtggacctgctgttcaagaccaacagaaaagtgaccgtgaagcagctgaaagaggactacttcaagaaaatcgagtgcttcgactccgtggaaatctccggcgtggaagatagattcaacgcctccctgggcacataccacgatctgctgaaaattatcaaggacaaggacttcctggataacgaagagaacgaggacattctggaagatatcgtgctgaccctgacactgtttgaggaccgcgagatgatcgaggaaaggctgaaaacctacgctcacctgttcgacgacaaagtgatgaagcagctgaagagaaggcggtacaccggctggggcaggctgagcagaaagctgatcaacggcatcagagacaagcagagcggcaagacaatcctggatttcctgaagtccgacggcttcgccaaccggaacttcatgcagctgatccacgacgacagcctgacattcaaagaggacatccagaaagcccaggtgtccggccagggcgactctctgcacgagcatatcgctaacctggccggcagccccgctatcaagaagggcatcctgcagacagtgaaggtggtggacgagctcgtgaaagtgatgggcagacacaagcccgagaacatcgtgatcgagatggctagagagaaccagaccacccagaagggacagaagaactcccgcgagaggatgaagagaatcgaagagggcatcaaagagctgggcagccagatcctgaaagaacaccccgtggaaaacacccagctgcagaacgagaagctgtacctgtactacctgcagaatggccgggatatgtacgtggaccaggaactggacatcaacagactgtccgactacgatgtggaccatatcgtgcctcagagctttctgaaggacgactccatcgataacaaagtgctgactcggagcgacaagaacagaggcaagagcgacaacgtgccctccgaagaggtcgtgaagaagatgaagaactactggcgacagctgctgaacgccaagctgattacccagaggaagttcgataacctgaccaaggccgagagaggcggcctgagcgagctggataaggccggcttcatcaagaggcagctggtggaaaccagacagatcacaaagcacgtggcacagatcctggactcccggatgaacactaagtacgacgaaaacgataagctgatccgggaagtgaaagtgatcaccctgaagtccaagctggtgtccgatttccggaaggatttccagttttacaaagtgcgcgagatcaacaactaccaccacgcccacgacgcctacctgaacgccgtcgtgggaaccgccctgatcaaaaagtaccctaagctggaaagcgagttcgtgtacggcgactacaaggtgtacgacgtgcggaagatgatcgccaagagcgagcaggaaatcggcaaggctaccgccaagtacttcttctacagcaacatcatgaactttttcaagaccgaaatcaccctggccaacggcgagatcagaaagcgccctctgatcgagacaaacggcgaaaccggggagatcgtgtgggataagggcagagacttcgccacagtgcgaaaggtgctgagcatgccccaagtgaatatcgtgaaaaagaccgaggtgcagacaggcggcttcagcaaagagtctatcctgcccaagaggaacagcgacaagctgatcgccagaaagaaggactgggaccccaagaagtacggcggcttcgacagccctaccgtggcctactctgtgctggtggtggctaaggtggaaaagggcaagtccaagaaactgaagagtgtgaaagagctgctggggatcaccatcatggaaagaagcagctttgagaagaaccctatcgactttctggaagccaagggctacaaagaagtgaaaaaggacctgatcatcaagctgcctaagtactccctgttcgagctggaaaacggcagaaagagaatgctggcctctgccggcgaactgcagaagggaaacgagctggccctgcctagcaaatatgtgaacttcctgtacctggcctcccactatgagaagctgaagggcagccctgaggacaacgaacagaaacagctgtttgtggaacagcataagcactacctggacgagatcatcgagcagatcagcgagttctccaagagagtgatcctggccgacgccaatctggacaaggtgctgtctgcctacaacaagcacagggacaagcctatcagagagcaggccgagaatatcatccacctgttcaccctgacaaacctgggcgctcctgccgccttcaagtactttgacaccaccatcgaccggaagaggtacaccagcaccaaagaggtgctggacgccaccctgatccaccagagcatcaccggcctgtacgagacaagaatcgacctgtctcagctgggaggcgacaagagacctgccgccactaagaaggccggacaggccaaaaagaagaagtga

SEQ ID NO: 94 - protein, 1391 aa, synthetic construct
  REGION 1..1391: note = Synthetic
  REGION 4..10: note = MISC_FEATURE - 5' NLS
  REGION 1376..1391: note = MISC_FEATURE - 3' NLS
MDKPKKKRKVKYSIGLDIGTNSVGWAVITDEYKVPSKKFKVLGNTDRHSIKKNLIGALLFDSGETAEATRLKRTARRRYTRRKNRICYLQEIFSNEMAKVDDSFFHRLEESFLVEEDKKHERHPIFGNIVDEVAYHEKYPTIYHLRKKLVDSTDKADLRLIYLALAHMIKFRGHFLIEGDLNPDNSDVDKLFIQLVQTYNQLFEENPINASGVDAKAILSARLSKSRRLENLIAQLPGEKKNGLFGNLIALSLGLTPNFKSNFDLAEDAKLQLSKDTYDDDLDNLLAQIGDQYADLFLAAKNLSDAILLSDILRVNTEITKAPLSASMIKRYDEHHQDLTLLKALVRQQLPEKYKEIFFDQSKNGYAGYIDGGASQEEFYKFIKPILEKMDGTEELLVKLNREDLLRKQRTFDNGSIPHQIHLGELHAILRRQEDFYPFLKDNREKIEKILTFRIPYYVGPLARGNSRFAWMTRKSEETITPWNFEEVVDKGASAQSFIERMTNFDKNLPNEKVLPKHSLLYEYFTVYNELTKVKYVTEGMRKPAFLSGEQKKAIVDLLFKTNRKVTVKQLKEDYFKKIECFDSVEISGVEDRFNASLGTYHDLLKIIKDKDFLDNEENEDILEDIVLTLTLFEDREMIEERLKTYAHLFDDKVMKQLKRRRYTGWGRLSRKLINGIRDKQSGKTILDFLKSDGFANRNFMQLIHDDSLTFKEDIQKAQVSGQGDSLHEHIANLAGSPAIKKGILQTVKVVDELVKVMGRHKPENIVIEMARENQTTQKGQKNSRERMKRIEEGIKELGSQILKEHPVENTQLQNEKLYLYYLQNGRDMYVDQELDINRLSDYDVDHIVPQSFLKDDSIDNKVLTRSDKNRGKSDNVPSEEVVKKMKNYWRQLLNAKLITQRKFDNLTKAERGGLSELDKAGFIKRQLVETRQITKHVAQILDSRMNTKYDENDKLIREVKVITLKSKLVSDFRKDFQFYKVREINNYHHAHDAYLNAVVGTALIKKYPKLESEFVYGDYKVYDVRKMIAKSEQEIGKATAKYFFYSNIMNFFKTEITLANGEIRKRPLIETNGETGEIVWDKGRDFATVRKVLSMPQVNIVKKTEVQTGGFSKESILPKRNSDKLIARKKDWDPKKYGGFDSPTVAYSVLVVAKVEKGKSKKLKSVKELLGITIMERSSFEKNPIDFLEAKGYKEVKKDLIIKLPKYSLFELENGRKRMLASAGELQKGNELALPSKYVNFLYLASHYEKLKGSPEDNEQKQLFVEQHKHYLDEIIEQISEFSKRVILADANLDKVLSAYNKHRDKPIREQAENIIHLFTLTNLGAPAAFKYFDTTIDRKRYTSTKEVLDATLIHQSITGLYETRIDLSQLGGDKRPAATKKAGQAKKKK